European Patent Application EP 4 134 433 A1, published February 15, 2023. Title: SERPINA1 SIRNAS: COMPOSITIONS OF MATTER AND METHODS OF TREATMENT. Applicant: ALNYLAM PHARMACEUTICALS, INC. The sequence listing filed with the application follows.

SEQUENCE LISTING (204 sequences)

SEQ ID NO: 1 - DNA, 3220 bp, Homo sapiens
acaatgactcctttcggtaagtgcagtggaagctgtacactgcccaggcaaagcgtccgggcagcgtaggcgggcgactcagatcccagccagtggacttagcccctgtttgctcctccgataactggggtgaccttggttaatattcaccagcagcctcccccgttgcccctctggatccactgcttaaatacggacgaggacagggccctgtctcctcagcttcaggcaccaccactgacctgggacagtgaatcgacaatgccgtcttctgtctcgtggggcatcctcctgctggcaggcctgtgctgcctggtccctgtctccctggctgaggatccccagggagatgctgcccagaagacagatacatcccaccatgatcaggatcacccaaccttcaacaagatcacccccaacctggctgagttcgccttcagcctataccgccagctggcacaccagtccaacagcaccaatatcttcttctccccagtgagcatcgctacagcctttgcaatgctctccctggggaccaaggctgacactcacgatgaaatcctggagggcctgaatttcaacctcacggagattccggaggctcagatccatgaaggcttccaggaactcctccgtaccctcaaccagccagacagccagctccagctgaccaccggcaatggcctgttcctcagcgagggcctgaagctagtggataagtttttggaggatgttaaaaagttgtaccactcagaagccttcactgtcaacttcggggacaccgaagaggccaagaaacagatcaacgattacgtggagaagggtactcaagggaaaattgtggatttggtcaaggagcttgacagagacacagtttttgctctggtgaattacatcttctttaaaggcaaatgggagagaccctttgaagtcaaggacaccgaggaagaggacttccacgtggaccaggtgaccaccgtgaaggtgcctatgatgaagcgtttaggcatgtttaacatccagcactgtaagaagctgtccagctgggtgctgctgatgaaatacctgggcaatgccaccgccatcttcttcctgcctgatgaggggaaactacagcacctggaaaatgaactcacccacgatatcatcaccaagttcctggaaaatgaagacagaaggtctgccagcttacatttacccaaactgtccattactggaacctatgatctgaagagcgtcctgggtcaactgggcatcactaaggtcttcagcaatggggctgacctctccggggtcacagaggaggcacccctgaagctctccaaggccgtgcataaggctgtgctgaccatcgacgagaaagggactgaagctgctggggccatgtttttagaggccatacccatgtctatcccccccgaggtcaagttcaacaaaccctttgtcttcttaatgattgaacaaaataccaagtctcccctcttcatgggaaaagtggtgaatcccacccaaaaataactgcctctcgctcctcaacccctcccctccatccctggccccctccctggatgacattaaagaagggttgagctggtccctgcctgcatgtgactgtaaatccctcccatgttttctctgagtctccctttgcctgctgaggctgtatgtgggctccaggtaacagtgctgtcttcgggccccctgaactgtgttcatggagcatctggctgggtaggcacatgctgggcttgaatccaggggggactgaatcctcagcttacggacctgggcccatctgtttctggagggctccagtcttccttgtcctgtcttggagtccccaagaaggaatcacaggggaggaaccagataccagccatgaccccaggctccaccaagcatcttcatgtccccctgctcatcccccactcccccccacccagagttgctcatcctgccagggctggctgtgcccaccccaaggctgccctcctgggggccccagaactgcctgatcgtgccgtggcccagttttgtggcatctgcagcaacacaagagagaggacaatgtcctcctcttgacccgctgtcacctaaccagactcgggccctgcacctctcaggcacttctggaaaatgactgaggcagattcttcctgaagcccattctccatggggcaacaaggacacctattctgtccttgtccttccatcgctgccccagaaagcctcacatatctccgtttagaatcaggtcccttctccccagatgaagaggagggtctctgctttgttttctctatctcctcctcagacttgaccaggcccagcaggccccagaagaccattaccctatatcccttctcctccctagtcacatggccataggcctgctgatggctcaggaaggccattgcaaggactcctcagctatgggagaggaagcacatcacccattgacccccgcaacccctccctttcctcctctgagtcccgactggggccacatgcagcctgacttctttgtgcctgttgctgtccctgcagtcttcagagggccaccgcagctccagtgccacggcaggaggctgttcctgaatagcccctgtggtaagggccaggagagtccttccatcctccaaggccctgctaaaggacacagcagccaggaagtcccctgggcccctagctgaaggacagcctgctccctccgtctctaccaggaatggccttgtcctatggaaggcactgccccatcccaaactaatctaggaatcactgtctaaccactcactgtcatgaatgtgtacttaaaggatgaggttgagtcataccaaatagtgatttcgatagttcaaaatggtgaaattagcaattctacatgattcagtctaatcaatggataccgactgtttcccacacaagtctcctgttctcttaagcttactcactgacagcctttcactctccacaaatacattaaagatatggccatcaccaagccccctaggatgacaccagacctgagagtctgaagacctggatccaagttctgacttttccccctgacagctgtgtgaccttcgtgaagtcgccaaacctctctgagccccagtcattgctagtaagacctgcctttgagttggtatgatgttcaagttagataacaaaatgtttatacccattagaacagagaataaatagaactacatttcttgca

SEQ ID NO: 2 - DNA, 3199 bp, Homo sapiens
tgggcaggaactgggcactgtgcccagggcatgcactgcctccacgcagcaaccctcagagtcctgagctgaaccaagaaggaggagggggtcgggcctccgaggaaggcctagccgctgctgctgccaggaattccaggttggaggggcggcaacctcctgccagccttcaggccactctcctgtgcctgccagaagagacagagcttgaggagagcttgaggagagcaggaaaggacaatgccgtcttctgtctcgtggggcatcctcctgctggcaggcctgtgctgcctggtccctgtctccctggctgaggatccccagggagatgctgcccagaagacagatacatcccaccatgatcaggatcacccaaccttcaacaagatcacccccaacctggctgagttcgccttcagcctataccgccagctggcacaccagtccaacagcaccaatatcttcttctccccagtgagcatcgctacagcctttgcaatgctctccctggggaccaaggctgacactcacgatgaaatcctggagggcctgaatttcaacctcacggagattccggaggctcagatccatgaaggcttccaggaactcctccgtaccctcaaccagccagacagccagctccagctgaccaccggcaatggcctgttcctcagcgagggcctgaagctagtggataagtttttggaggatgttaaaaagttgtaccactcagaagccttcactgtcaacttcggggacaccgaagaggccaagaaacagatcaacgattacgtggagaagggtactcaagggaaaattgtggatttggtcaaggagcttgacagagacacagtttttgctctggtgaattacatcttctttaaaggcaaatgggagagaccctttgaagtcaaggacaccgaggaagaggacttccacgtggaccaggtgaccaccgtgaaggtgcctatgatgaagcgtttaggcatgtttaacatccagcactgtaagaagctgtccagctgggtgctgctgatgaaatacctgggcaatgccaccgccatcttcttcctgcctgatgaggggaaactacagcacctggaaaatgaactcacccacgatatcatcaccaagttcctggaaaatgaagacagaaggtctgccagcttacatttacccaaactgtccattactggaacctatgatctgaagagcgtcctgggtcaactgggcatcactaaggtcttcagcaatggggctgacctctccggggtcacagaggaggcacccctgaagctctccaaggccgtgcataaggctgtgctgaccatcgacgagaaagggactgaagctgctggggccatgtttttagaggccatacccatgtctatcccccccgaggtcaagttcaacaaaccctttgtcttcttaatgattgaacaaaataccaagtctcccctcttcatgggaaaagtggtgaatcccacccaaaaataactgcctctcgctcctcaacccctcccctccatccctggccccctccctggatgacattaaagaagggttgagctggtccctgcctgcatgtgactgtaaatccctcccatgttttctctgagtctccctttgcctgctgaggctgtatgtgggctccaggtaacagtgctgtcttcgggccccctgaactgtgttcatggagcatctggctgggtaggcacatgctgggcttgaatccaggggggactgaatcctcagcttacggacctgggcccatctgtttctggagggctccagtcttccttgtcctgtcttggagtccccaagaaggaatcacaggggaggaaccagataccagccatgaccccaggctccaccaagcatcttcatgtccccctgctcatcccccactcccccccacccagagttgctcatcctgccagggctggctgtgcccaccccaaggctgccctcctgggggccccagaactgcctgatcgtgccgtggcccagttttgtggcatctgcagcaacacaagagagaggacaatgtcctcctcttgacccgctgtcacctaaccagactcgggccctgcacctctcaggcacttctggaaaatgactgaggcagattcttcctgaagcccattctccatggggcaacaaggacacctattctgtccttgtccttccatcgctgccccagaaagcctcacatatctccgtttagaatcaggtcccttctccccagatgaagaggagggtctctgctttgttttctctatctcctcctcagacttgaccaggcccagcaggccccagaagaccattaccctatatcccttctcctccctagtcacatggccataggcctgctgatggctcaggaaggccattgcaaggactcctcagctatgggagaggaagcacatcacccattgacccccgcaacccctccctttcctcctctgagtcccgactggggccacatgcagcctgacttctttgtgcctgttgctgtccctgcagtcttcagagggccaccgcagctccagtgccacggcaggaggctgttcctgaatagcccctgtggtaagggccaggagagtccttccatcctccaaggccctgctaaaggacacagcagccaggaagtcccctgggcccctagctgaaggacagcctgctccctccgtctctaccaggaatggccttgtcctatggaaggcactgccccatcccaaactaatctaggaatcactgtctaaccactcactgtcatgaatgtgtacttaaaggatgaggttgagtcataccaaatagtgatttcgatagttcaaaatggtgaaattagcaattctacatgattcagtctaatcaatggataccgactgtttcccacacaagtctcctgttctcttaagcttactcactgacagcctttcactctccacaaatacattaaagatatggccatcaccaagccccctaggatgacaccagacctgagagtctgaagacctggatccaagttctgacttttccccctgacagctgtgtgaccttcgtgaagtcgccaaacctctctgagccccagtcattgctagtaagacctgcctttgagttggtatgatgttcaagttagataacaaaatgtttatacccattagaacagagaataaatagaactacatttcttgca

SEQ ID NO: 3 - DNA, 3513 bp, Homo sapiens
tgggcaggaactgggcactgtgcccagggcatgcactgcctccacgcagcaaccctcagagtcctgagctgaaccaagaaggaggagggggtcgggcctccgaggaaggcctagccgctgctgctgccaggaattccaggttggaggggcggcaacctcctgccagccttcaggccactctcctgtgcctgccagaagagacagagcttgaggagagcttgaggagagcaggaaagggcggcagtaagtcttcagcatcaggcattttggggtgactcagtaaatggtagatcttgctaccagtggaacagccactaaggattctgcagtgagagcagagggccagctaagtggtactctcccagagactgtctgactcacgccaccccctccaccttggacacaggacgctgtggtttctgagccaggtacaatgactcctttcgcagcctcccccgttgcccctctggatccactgcttaaatacggacgaggacagggccctgtctcctcagcttcaggcaccaccactgacctgggacagtgaatcgacaatgccgtcttctgtctcgtggggcatcctcctgctggcaggcctgtgctgcctggtccctgtctccctggctgaggatccccagggagatgctgcccagaagacagatacatcccaccatgatcaggatcacccaaccttcaacaagatcacccccaacctggctgagttcgccttcagcctataccgccagctggcacaccagtccaacagcaccaatatcttcttctccccagtgagcatcgctacagcctttgcaatgctctccctggggaccaaggctgacactcacgatgaaatcctggagggcctgaatttcaacctcacggagattccggaggctcagatccatgaaggcttccaggaactcctccgtaccctcaaccagccagacagccagctccagctgaccaccggcaatggcctgttcctcagcgagggcctgaagctagtggataagtttttggaggatgttaaaaagttgtaccactcagaagccttcactgtcaacttcggggacaccgaagaggccaagaaacagatcaacgattacgtggagaagggtactcaagggaaaattgtggatttggtcaaggagcttgacagagacacagtttttgctctggtgaattacatcttctttaaaggcaaatgggagagaccctttgaagtcaaggacaccgaggaagaggacttccacgtggaccaggtgaccaccgtgaaggtgcctatgatgaagcgtttaggcatgtttaacatccagcactgtaagaagctgtccagctgggtgctgctgatgaaatacctgggcaatgccaccgccatcttcttcctgcctgatgaggggaaactacagcacctggaaaatgaactcacccacgatatcatcaccaagttcctggaaaatgaagacagaaggtctgccagcttacatttacccaaactgtccattactggaacctatgatctgaagagcgtcctgggtcaactgggcatcactaaggtcttcagcaatggggctgacctctccggggtcacagaggaggcacccctgaagctctccaaggccgtgcataaggctgtgctgaccatcgacgagaaagggactgaagctgctggggccatgtttttagaggccatacccatgtctatcccccccgaggtcaagttcaacaaaccctttgtcttcttaatgattgaacaaaataccaagtctcccctcttcatgggaaaagtggtgaatcccacccaaaaataactgcctctcgctcctcaacccctcccctccatccctggccccctccctggatgacattaaagaagggttgagctggtccctgcctgcatgtgactgtaaatccctcccatgttttctctgagtctccctttgcctgctgaggctgtatgtgggctccaggtaacagtgctgtcttcgggccccctgaactgtgttcatggagcatctggctgggtaggcacatgctgggcttgaatccaggggggactgaatcctcagcttacggacctgggcccatctgtttctggagggctccagtcttccttgtcctgtcttggagtccccaagaaggaatcacaggggaggaaccagataccagccatgaccccaggctccaccaagcatcttcatgtccccctgctcatcccccactcccccccacccagagttgctcatcctgccagggctggctgtgcccaccccaaggctgccctcctgggggccccagaactgcctgatcgtgccgtggcccagttttgtggcatctgcagcaacacaagagagaggacaatgtcctcctcttgacccgctgtcacctaaccagactcgggccctgcacctctcaggcacttctggaaaatgactgaggcagattcttcctgaagcccattctccatggggcaacaaggacacctattctgtccttgtccttccatcgctgccccagaaagcctcacatatctccgtttagaatcaggtcccttctccccagatgaagaggagggtctctgctttgttttctctatctcctcctcagacttgaccaggcccagcaggccccagaagaccattaccctatatcccttctcctccctagtcacatggccataggcctgctgatggctcaggaaggccattgcaaggactcctcagctatgggagaggaagcacatcacccattgacccccgcaacccctccctttcctcctctgagtcccgactggggccacatgcagcctgacttctttgtgcctgttgctgtccctgcagtcttcagagggccaccgcagctccagtgccacggcaggaggctgttcctgaatagcccctgtggtaagggccaggagagtccttccatcctccaaggccctgctaaaggacacagcagccaggaagtcccctgggcccctagctgaaggacagcctgctccctccgtctctaccaggaatggccttgtcctatggaaggcactgccccatcccaaactaatctaggaatcactgtctaaccactcactgtcatgaatgtgtacttaaaggatgaggttgagtcataccaaatagtgatttcgatagttcaaaatggtgaaattagcaattctacatgattcagtctaatcaatggataccgactgtttcccacacaagtctcctgttctcttaagcttactcactgacagcctttcactctccacaaatacattaaagatatggccatcaccaagccccctaggatgacaccagacctgagagtctgaagacctggatccaagttctgacttttccccctgacagctgtgtgaccttcgtgaagtcgccaaacctctctgagccccagtcattgctagtaagacctgcctttgagttggtatgatgttcaagttagataacaaaatgtttatacccattagaacagagaataaatagaactacatttcttgca

SEQ ID NO: 4 - DNA, 3236 bp, Homo sapiens
tgggcaggaactgggcactgtgcccagggcatgcactgcctccacgcagcaaccctcagagtcctgagctgaaccaagaaggaggagggggtcgggcctccgaggaaggcctagccgctgctgctgccaggaattccaggttggaggggcggcaacctcctgccagccttcaggccactctcctgtgcctgccagaagagacagagcttgaggagagcttgaggagagcaggaaaggtgggacattgctgctgctgctcactcagttccacaggacaatgccgtcttctgtctcgtggggcatcctcctgctggcaggcctgtgctgcctggtccctgtctccctggctgaggatccccagggagatgctgcccagaagacagatacatcccaccatgatcaggatcacccaaccttcaacaagatcacccccaacctggctgagttcgccttcagcctataccgccagctggcacaccagtccaacagcaccaatatcttcttctccccagtgagcatcgctacagcctttgcaatgctctccctggggaccaaggctgacactcacgatgaaatcctggagggcctgaatttcaacctcacggagattccggaggctcagatccatgaaggcttccaggaactcctccgtaccctcaaccagccagacagccagctccagctgaccaccggcaatggcctgttcctcagcgagggcctgaagctagtggataagtttttggaggatgttaaaaagttgtaccactcagaagccttcactgtcaacttcggggacaccgaagaggccaagaaacagatcaacgattacgtggagaagggtactcaagggaaaattgtggatttggtcaaggagcttgacagagacacagtttttgctctggtgaattacatcttctttaaaggcaaatgggagagaccctttgaagtcaaggacaccgaggaagaggacttccacgtggaccaggtgaccaccgtgaaggtgcctatgatgaagcgtttaggcatgtttaacatccagcactgtaagaagctgtccagctgggtgctgctgatgaaatacctgggcaatgccaccgccatcttcttcctgcctgatgaggggaaactacagcacctggaaaatgaactcacccacgatatcatcaccaagttcctggaaaatgaagacagaaggtctgccagcttacatttacccaaactgtccattactggaacctatgatctgaagagcgtcctgggtcaactgggcatcactaaggtcttcagcaatggggctgacctctccggggtcacagaggaggcacccctgaagctctccaaggccgtgcataaggctgtgctgaccatcgacgagaaagggactgaagctgctggggccatgtttttagaggccatacccatgtctatcccccccgaggtcaagttcaacaaaccctttgtcttcttaatgattgaacaaaataccaagtctcccctcttcatgggaaaagtggtgaatcccacccaaaaataactgcctctcgctcctcaacccctcccctccatccctggccccctccctggatgacattaaagaagggttgagctggtccctgcctgcatgtgactgtaaatccctcccatgttttctctgagtctccctttgcctgctgaggctgtatgtgggctccaggtaacagtgctgtcttcgggccccctgaactgtgttcatggagcatctggctgggtaggcacatgctgggcttgaatccaggggggactgaatcctcagcttacggacctgggcccatctgtttctggagggctccagtcttccttgtcctgtcttggagtccccaagaaggaatcacaggggaggaaccagataccagccatgaccccaggctccaccaagcatcttcatgtccccctgctcatcccccactcccccccacccagagttgctcatcctgccagggctggctgtgcccaccccaaggctgccctcctgggggccccagaactgcctgatcgtgccgtggcccagttttgtggcatctgcagcaacacaagagagaggacaatgtcctcctcttgacccgctgtcacctaaccagactcgggccctgcacctctcaggcacttctggaaaatgactgaggcagattcttcctgaagcccattctccatggggcaacaaggacacctattctgtccttgtccttccatcgctgccccagaaagcctcacatatctccgtttagaatcaggtcccttctccccagatgaagaggagggtctctgctttgttttctctatctcctcctcagacttgaccaggcccagcaggccccagaagaccattaccctatatcccttctcctccctagtcacatggccataggcctgctgatggctcaggaaggccattgcaaggactcctcagctatgggagaggaagcacatcacccattgacccccgcaacccctccctttcctcctctgagtcccgactggggccacatgcagcctgacttctttgtgcctgttgctgtccctgcagtcttcagagggccaccgcagctccagtgccacggcaggaggctgttcctgaatagcccctgtggtaagggccaggagagtccttccatcctccaaggccctgctaaaggacacagcagccaggaagtcccctgggcccctagctgaaggacagcctgctccctccgtctctaccaggaatggccttgtcctatggaaggcactgccccatcccaaactaatctaggaatcactgtctaaccactcactgtcatgaatgtgtacttaaaggatgaggttgagtcataccaaatagtgatttcgatagttcaaaatggtgaaattagcaattctacatgattcagtctaatcaatggataccgactgtttcccacacaagtctcctgttctcttaagcttactcactgacagcctttcactctccacaaatacattaaagatatggccatcaccaagccccctaggatgacaccagacctgagagtctgaagacctggatccaagttctgacttttccccctgacagctgtgtgaccttcgtgaagtcgccaaacctctctgagccccagtcattgctagtaagacctgcctttgagttggtatgatgttcaagttagataacaaaatgtttatacccattagaacagagaataaatagaactacatttcttgca

SEQ ID NO: 5 - DNA, 3532 bp, Homo sapiens
tgggcaggaactgggcactgtgcccagggcatgcactgcctccacgcagcaaccctcagagtcctgagctgaaccaagaaggaggagggggtcgggcctccgaggaaggcctagccgctgctgctgccaggaattccaggttggaggggcggcaacctcctgccagccttcaggccactctcctgtgcctgccagaagagacagagcttgaggagagcttgaggagagcaggaaaggtgggacattgctgctgctgctcactcagttccacagggcggcagtaagtcttcagcatcaggcattttggggtgactcagtaaatggtagatcttgctaccagtggaacagccactaaggattctgcagtgagagcagagggccagctaagtggtactctcccagagactgtctgactcacgccaccccctccaccttggacacaggacgctgtggtttctgagccagcagcctcccccgttgcccctctggatccactgcttaaatacggacgaggacagggccctgtctcctcagcttcaggcaccaccactgacctgggacagtgaatcgacaatgccgtcttctgtctcgtggggcatcctcctgctggcaggcctgtgctgcctggtccctgtctccctggctgaggatccccagggagatgctgcccagaagacagatacatcccaccatgatcaggatcacccaaccttcaacaagatcacccccaacctggctgagttcgccttcagcctataccgccagctggcacaccagtccaacagcaccaatatcttcttctccccagtgagcatcgctacagcctttgcaatgctctccctggggaccaaggctgacactcacgatgaaatcctggagggcctgaatttcaacctcacggagattccggaggctcagatccatgaaggcttccaggaactcctccgtaccctcaaccagccagacagccagctccagctgaccaccggcaatggcctgttcctcagcgagggcctgaagctagtggataagtttttggaggatgttaaaaagttgtaccactcagaagccttcactgtcaacttcggggacaccgaagaggccaagaaacagatcaacgattacgtggagaagggtactcaagggaaaattgtggatttggtcaaggagcttgacagagacacagtttttgctctggtgaattacatcttctttaaaggcaaatgggagagaccctttgaagtcaaggacaccgaggaagaggacttccacgtggaccaggtgaccaccgtgaaggtgcctatgatgaagcgtttaggcatgtttaacatccagcactgtaagaagctgtccagctgggtgctgctgatgaaatacctgggcaatgccaccgccatcttcttcctgcctgatgaggggaaactacagcacctggaaaatgaactcacccacgatatcatcaccaagttcctggaaaatgaagacagaaggtctgccagcttacatttacccaaactgtccattactggaacctatgatctgaagagcgtcctgggtcaactgggcatcactaaggtcttcagcaatggggctgacctctccggggtcacagaggaggcacccctgaagctctccaaggccgtgcataaggctgtgctgaccatcgacgagaaagggactgaagctgctggggccatgtttttagaggccatacccatgtctatcccccccgaggtcaagttcaacaaaccctttgtcttcttaatgattgaacaaaataccaagtctcccctcttcatgggaaaagtggtgaatcccacccaaaaataactgcctctcgctcctcaacccctcccctccatccctggccccctccctggatgacattaaagaagggttgagctggtccctgcctgcatgtgactgtaaatccctcccatgttttctctgagtctccctttgcctgctgaggctgtatgtgggctccaggtaacagtgctgtcttcgggccccctgaactgtgttcatggagcatctggctgggtaggcacatgctgggcttgaatccaggggggactgaatcctcagcttacggacctgggcccatctgtttctggagggctccagtcttccttgtcctgtcttggagtccccaagaaggaatcacaggggaggaaccagataccagccatgaccccaggctccaccaagcatcttcatgtccccctgctcatcccccactcccccccacccagagttgctcatcctgccagggctggctgtgcccaccccaaggctgccctcctgggggccccagaactgcctgatcgtgccgtggcccagttttgtggcatctgcagcaacacaagagagaggacaatgtcctcctcttgacccgctgtcacctaaccagactcgggccctgcacctctcaggcacttctggaaaatgactgaggcagattcttcctgaagcccattctccatggggcaacaaggacacctattctgtccttgtccttccatcgctgccccagaaagcctcacatatctccgtttagaatcaggtcccttctccccagatgaagaggagggtctctgctttgttttctctatctcctcctcagacttgaccaggcccagcaggccccagaagaccattaccctatatcccttctcctccctagtcacatggccataggcctgctgatggctcaggaaggccattgcaaggactcctcagctatgggagaggaagcacatcacccattgacccccgcaacccctccctttcctcctctgagtcccgactggggccacatgcagcctgacttctttgtgcctgttgctgtccctgcagtcttcagagggccaccgcagctccagtgccacggcaggaggctgttcctgaatagcccctgtggtaagggccaggagagtccttccatcctccaaggccctgctaaaggacacagcagccaggaagtcccctgggcccctagctgaaggacagcctgctccctccgtctctaccaggaatggccttgtcctatggaaggcactgccccatcccaaactaatctaggaatcactgtctaaccactcactgtcatgaatgtgtacttaaaggatgaggttgagtcataccaaatagtgatttcgatagttcaaaatggtgaaattagcaattctacatgattcagtctaatcaatggataccgactgtttcccacacaagtctcctgttctcttaagcttactcactgacagcctttcactctccacaaatacattaaagatatggccatcaccaagccccctaggatgacaccagacctgagagtctgaagacctggatccaagttctgacttttccccctgacagctgtgtgaccttcgtgaagtcgccaaacctctctgagccccagtcattgctagtaagacctgcctttgagttggtatgatgttcaagttagataacaaaatgtttatacccattagaacagagaataaatagaactacatttcttgca

SEQ ID NO: 6 - DNA, 3340 bp, Homo sapiens
tgggcaggaactgggcactgtgcccagggcatgcactgcctccacgcagcaaccctcagagtcctgagctgaaccaagaaggaggagggggtcgggcctccgaggaaggcctagccgctgctgctgccaggaattccaggttggaggggcggcaacctcctgccagccttcaggccactctcctgtgcctgccagaagagacagagcttgaggagagcttgaggagagcaggaaaggtgggacattgctgctgctgctcactcagttccacagcagcctcccccgttgcccctctggatccactgcttaaatacggacgaggacagggccctgtctcctcagcttcaggcaccaccactgacctgggacagtgaatcgacaatgccgtcttctgtctcgtggggcatcctcctgctggcaggcctgtgctgcctggtccctgtctccctggctgaggatccccagggagatgctgcccagaagacagatacatcccaccatgatcaggatcacccaaccttcaacaagatcacccccaacctggctgagttcgccttcagcctataccgccagctggcacaccagtccaacagcaccaatatcttcttctccccagtgagcatcgctacagcctttgcaatgctctccctggggaccaaggctgacactcacgatgaaatcctggagggcctgaatttcaacctcacggagattccggaggctcagatccatgaaggcttccaggaactcctccgtaccctcaaccagccagacagccagctccagctgaccaccggcaatggcctgttcctcagcgagggcctgaagctagtggataagtttttggaggatgttaaaaagttgtaccactcagaagccttcactgtcaacttcggggacaccgaagaggccaagaaacagatcaacgattacgtggagaagggtactcaagggaaaattgtggatttggtcaaggagcttgacagagacacagtttttgctctggtgaattacatcttctttaaaggcaaatgggagagaccctttgaagtcaaggacaccgaggaagaggacttccacgtggaccaggtgaccaccgtgaaggtgcctatgatgaagcgtttaggcatgtttaacatccagcactgtaagaagctgtccagctgggtgctgctgatgaaatacctgggcaatgccaccgccatcttcttcctgcctgatgaggggaaactacagcacctggaaaatgaactcacccacgatatcatcaccaagttcctggaaaatgaagacagaaggtctgccagcttacatttacccaaactgtccattactggaacctatgatctgaagagcgtcctgggtcaactgggcatcactaaggtcttcagcaatggggctgacctctccggggtcacagaggaggcacccctgaagctctccaaggccgtgcataaggctgtgctgaccatcgacgagaaagggactgaagctgctggggccatgtttttagaggccatacccatgtctatcccccccgaggtcaagttcaacaaaccctttgtcttcttaatgattgaacaaaataccaagtctcccctcttcatgggaaaagtggtgaatcccacccaaaaataactgcctctcgctcctcaacccctcccctccatccctggccccctccctggatgacattaaagaagggttgagctggtccctgcctgcatgtgactgtaaatccctcccatgttttctctgagtctccctttgcctgctgaggctgtatgtgggctccaggtaacagtgctgtcttcgggccccctgaactgtgttcatggagcatctggctgggtaggcacatgctgggcttgaatccaggggggactgaatcctcagcttacggacctgggcccatctgtttctggagggctccagtcttccttgtcctgtcttggagtccccaagaaggaatcacaggggaggaaccagataccagccatgaccccaggctccaccaagcatcttcatgtccccctgctcatcccccactcccccccacccagagttgctcatcctgccagggctggctgtgcccaccccaaggctgccctcctgggggccccagaactgcctgatcgtgccgtggcccagttttgtggcatctgcagcaacacaagagagaggacaatgtcctcctcttgacccgctgtcacctaaccagactcgggccctgcacctctcaggcacttctggaaaatgactgaggcagattcttcctgaagcccattctccatggggcaacaaggacacctattctgtccttgtccttccatcgctgccccagaaagcctcacatatctccgtttagaatcaggtcccttctccccagatgaagaggagggtctctgctttgttttctctatctcctcctcagacttgaccaggcccagcaggccccagaagaccattaccctatatcccttctcctccctagtcacatggccataggcctgctgatggctcaggaaggccattgcaaggactcctcagctatgggagaggaagcacatcacccattgacccccgcaacccctccctttcctcctctgagtcccgactggggccacatgcagcctgacttctttgtgcctgttgctgtccctgcagtcttcagagggccaccgcagctccagtgccacggcaggaggctgttcctgaatagcccctgtggtaagggccaggagagtccttccatcctccaaggccctgctaaaggacacagcagccaggaagtcccctgggcccctagctgaaggacagcctgctccctccgtctctaccaggaatggccttgtcctatggaaggcactgccccatcccaaactaatctaggaatcactgtctaaccactcactgtcatgaatgtgtacttaaaggatgaggttgagtcataccaaatagtgatttcgatagttcaaaatggtgaaattagcaattctacatgattcagtctaatcaatggataccgactgtttcccacacaagtctcctgttctcttaagcttactcactgacagcctttcactctccacaaatacattaaagatatggccatcaccaagccccctaggatgacaccagacctgagagtctgaagacctggatccaagttctgacttttccccctgacagctgtgtgaccttcgtgaagtcgccaaacctctctgagccccagtcattgctagtaagacctgcctttgagttggtatgatgttcaagttagataacaaaatgtttatacccattagaacagagaataaatagaactacatttcttgca

SEQ ID NO: 7 - DNA, 3495 bp, Homo sapiens
tgggcaggaactgggcactgtgcccagggcatgcactgcctccacgcagcaaccctcagagtcctgagctgaaccaagaaggaggagggggtcgggcctccgaggaaggcctagccgctgctgctgccaggaattccaggttggaggggcggcaacctcctgccagccttcaggccactctcctgtgcctgccagaagagacagagcttgaggagagcttgaggagagcaggaaagggcggcagtaagtcttcagcatcaggcattttggggtgactcagtaaatggtagatcttgctaccagtggaacagccactaaggattctgcagtgagagcagagggccagctaagtggtactctcccagagactgtctgactcacgccaccccctccaccttggacacaggacgctgtggtttctgagccagcagcctcccccgttgcccctctggatccactgcttaaatacggacgaggacagggccctgtctcctcagcttcaggcaccaccactgacctgggacagtgaatcgacaatgccgtcttctgtctcgtggggcatcctcctgctggcaggcctgtgctgcctggtccctgtctccctggctgaggatccccagggagatgctgcccagaagacagatacatcccaccatgatcaggatcacccaaccttcaacaagatcacccccaacctggctgagttcgccttcagcctataccgccagctggcacaccagtccaacagcaccaatatcttcttctccccagtgagcatcgctacagcctttgcaatgctctccctggggaccaaggctgacactcacgatgaaatcctggagggcctgaatttcaacctcacggagattccggaggctcagatccatgaaggcttccaggaactcctccgtaccctcaaccagccagacagccagctccagctgaccaccggcaatggcctgttcctcagcgagggcctgaagctagtggataagtttttggaggatgttaaaaagttgtaccactcagaagccttcactgtcaacttcggggacaccgaagaggccaagaaacagatcaacgattacgtggagaagggtactcaagggaaaattgtggatttggtcaaggagcttgacagagacacagtttttgctctggtgaattacatcttctttaaaggcaaatgggagagaccctttgaagtcaaggacaccgaggaagaggacttccacgtggaccaggtgaccaccgtgaaggtgcctatgatgaagcgtttaggcatgtttaacatccagcactgtaagaagctgtccagctgggtgctgctgatgaaatacctgggcaatgccaccgccatcttcttcctgcctgatgaggggaaactacagcacctggaaaatgaactcacccacgatatcatcaccaagttcctggaaaatgaagacagaaggtctgccagcttacatttacccaaactgtccattactggaacctatgatctgaagagcgtcctgggtcaactgggcatcactaaggtcttcagcaatggggctgacctctccggggtcacagaggaggcacccctgaagctctccaaggccgtgcataaggctgtgctgaccatcgacgagaaagggactgaagctgctggggccatgtttttagaggccatacccatgtctatcccccccgaggtcaagttcaacaaaccctttgtcttcttaatgattgaacaaaataccaagtctcccctcttcatgggaaaagtggtgaatcccacccaaaaataactgcctctcgctcctcaacccctcccctccatccctggccccctccctggatgacattaaagaagggttgagctggtccctgcctgcatgtgactgtaaatccctcccatgttttctctgagtctccctttgcctgctgaggctgtatgtgggctccaggtaacagtgctgtcttcgggccccctgaactgtgttcatggagcatctggctgggtaggcacatgctgggcttgaatccaggggggactgaatcctcagcttacggacctgggcccatctgtttctggagggctccagtcttccttgtcctgtcttggagtccccaagaaggaatcacaggggaggaaccagataccagccatgaccccaggctccaccaagcatcttcatgtccccctgctcatcccccactcccccccacccagagttgctcatcctgccagggctggctgtgcccaccccaaggctgccctcctgggggccccagaactgcctgatcgtgccgtggcccagttttgtggcatctgcagcaacacaagagagaggacaatgtcctcctcttgacccgctgtcacctaaccagactcgggccctgcacctctcaggcacttctggaaaatgactgaggcagattcttcctgaagcccattctccatggggcaacaaggacacctattctgtccttgtccttccatcgctgccccagaaagcctcacatatctccgtttagaatcaggtcccttctccccagatgaagaggagggtctctgctttgttttctctatctcctcctcagacttgaccaggcccagcaggccccagaagaccattaccctatatcccttctcctccctagtcacatggccataggcctgctgatggctcaggaaggccattgcaaggactcctcagctatgggagaggaagcacatcacccattgacccccgcaacccctccctttcctcctctgagtcccgactggggccacatgcagcctgacttctttgtgcctgttgctgtccctgcagtcttcagagggccaccgcagctccagtgccacggcaggaggctgttcctgaatagcccctgtggtaagggccaggagagtccttccatcctccaaggccctgctaaaggacacagcagccaggaagtcccctgggcccctagctgaaggacagcctgctccctccgtctctaccaggaatggccttgtcctatggaaggcactgccccatcccaaactaatctaggaatcactgtctaaccactcactgtcatgaatgtgtacttaaaggatgaggttgagtcataccaaatagtgatttcgatagttcaaaatggtgaaattagcaattctacatgattcagtctaatcaatggataccgactgtttcccacacaagtctcctgttctcttaagcttactcactgacagcctttcactctccacaaatacattaaagatatggccatcaccaagccccctaggatgacaccagacctgagagtctgaagacctggatccaagttctgacttttccccctgacagctgtgtgaccttcgtgaagtcgccaaacctctctgagccccagtcattgctagtaagacctgcctttgagttggtatgatgttcaagttagataacaaaatgtttatacccattagaacagagaataaatagaactacatttcttgca

SEQ ID NO: 8 - DNA, 3492 bp, Homo sapiens
tgggcaggaactgggcactgtgcccagggcatgcactgcctccacgcagcaaccctcagagtcctgagctgaaccaagaaggaggagggggtcgggcctccgaggaaggcctagccgctgctgctgccaggaattccaggttggaggggcggcaacctcctgccagccttcaggccactctcctgtgcctgccagaagagacagagcttgaggagagcttgaggagagcaggaaagggcggcagtaagtcttcagcatcaggcattttggggtgactcagtaaatggtagatcttgctaccagtggaacagccactaaggattctgcagtgagagcagagggccagctaagtggtactctcccagagactgtctgactcacgccaccccctccaccttggacacaggacgctgtggtttctgagccagcctcccccgttgcccctctggatccactgcttaaatacggacgaggacagggccctgtctcctcagcttcaggcaccaccactgacctgggacagtgaatcgacaatgccgtcttctgtctcgtggggcatcctcctgctggcaggcctgtgctgcctggtccctgtctccctggctgaggatccccagggagatgctgcccagaagacagatacatcccaccatgatcaggatcacccaaccttcaacaagatcacccccaacctggctgagttcgccttcagcctataccgccagctggcacaccagtccaacagcaccaatatcttcttctccccagtgagcatcgctacagcctttgcaatgctctccctggggaccaaggctgacactcacgatgaaatcctggagggcctgaatttcaacctcacggagattccggaggctcagatccatgaaggcttccaggaactcctccgtaccctcaaccagccagacagccagctccagctgaccaccggcaatggcctgttcctcagcgagggcctgaagctagtggataagtttttggaggatgttaaaaagttgtaccactcagaagccttcactgtcaacttcggggacaccgaagaggccaagaaacagatcaacgattacgtggagaagggtactcaagggaaaattgtggatttggtcaaggagcttgacagagacacagtttttgctctggtgaattacatcttctttaaaggcaaatgggagagaccctttgaagtcaaggacaccgaggaagaggacttccacgtggaccaggtgaccaccgtgaaggtgcctatgatgaagcgtttaggcatgtttaacatccagcactgtaagaagctgtccagctgggtgctgctgatgaaatacctgggcaatgccaccgccatcttcttcctgcctgatgaggggaaactacagcacctggaaaatgaactcacccacgatatcatcaccaagttcctggaaaatgaagacagaaggtctgccagcttacatttacccaaactgtccattactggaacctatgatctgaagagcgtcctgggtcaactgggcatcactaaggtcttcagcaatggggctgacctctccggggtcacagaggaggcacccctgaagctctccaaggccgtgcataaggctgtgctgaccatcgacgagaaagggactgaagctgctggggccatgtttttagaggccatacccatgtctatcccccccgaggtcaagttcaacaaaccctttgtcttcttaatgattgaacaaaataccaagtctcccctcttcatgggaaaagtggtgaatcccacccaaaaataactgcctctcgctcctcaacccctcccctccatccctggccccctccctggatgacattaaagaagggttgagctggtccctgcctgcatgtgactgtaaatccctcccatgttttctctgagtctccctttgcctgctgaggctgtatgtgggctccaggtaacagtgctgtcttcgggccccctgaactgtgttcatggagcatctggctgggtaggcacatgctgggcttgaatccaggggggactgaatcctcagcttacggacctgggcccatctgtttctggagggctccagtcttccttgtcctgtcttggagtccccaagaaggaatcacaggggaggaaccagataccagccatgaccccaggctccaccaagcatcttcatgtccccctgctcatcccccactcccccccacccagagttgctcatcctgccagggctggctgtgcccaccccaaggctgccctcctgggggccccagaactgcctgatcgtgccgtggcccagttttgtggcatctgcagcaacacaagagagaggacaatgtcctcctcttgacccgctgtcacctaaccagactcgggccctgcacctctcaggcacttctggaaaatgactgaggcagattcttcctgaagcccattctccatggggcaacaaggacacctattctgtccttgtccttccatcgctgccccagaaagcctcacatatctccgtttagaatcaggtcccttctccccagatgaagaggagggtctctgctttgttttctctatctcctcctcagacttgaccaggcccagcaggccccagaagaccattaccctatatcccttctcctccctagtcacatggccataggcctgctgatggctcaggaaggccattgcaaggactcctcagctatgggagaggaagcacatcacccattgacccccgcaacccctccctttcctcctctgagtcccgactggggccacatgcagcctgacttctttgtgcctgttgctgtccctgcagtcttcagagggccaccgcagctccagtgccacggcaggaggctgttcctgaatagcccctgtggtaagggccaggagagtccttccatcctccaaggccctgctaaaggacacagcagccaggaagtcccctgggcccctagctgaaggacagcctgctccctccgtctctaccaggaatggccttgtcctatggaaggcactgccccatcccaaactaatctaggaatcactgtctaaccactcactgtcatgaatgtgtacttaaaggatgaggttgagtcataccaaatagtgatttcgatagttcaaaatggtgaaattagcaattctacatgattcagtctaatcaatggataccgactgtttcccacacaagtctcctgttctcttaagcttactcactgacagcctttcactctccacaaatacattaaagatatggccatcaccaagccccctaggatgacaccagacctgagagtctgaagacctggatccaagttctgacttttccccctgacagctgtgtgaccttcgtgaagtcgccaaacctctctgagccccagtcattgctagtaagacctgcctttgagttggtatgatgttcaagttagataacaaaatgtttatacccattagaacagagaataaatagaactacatttcttgca

SEQ ID NO: 9 - DNA, 3510 bp, Homo sapiens
tgggcaggaactgggcactgtgcccagggcatgcactgcctccacgcagcaaccctcagagtcctgagctgaaccaagaaggaggagggggtcgggcctccgaggaaggcctagccgctgctgctgccaggaattccaggttggaggggcggcaacctcctgccagccttcaggccactctcctgtgcctgccagaagagacagagcttgaggagagcttgaggagagcaggaaagggcggcagtaagtcttcagcatcaggcattttggggtgactcagtaaatggtagatcttgctaccagtggaacagccactaaggattctgcagtgagagcagagggccagctaagtggtactctcccagagactgtctgactcacgccaccccctccaccttggacacaggacgctgtggtttctgagccaggtacaatgactcctttcgcctcccccgttgcccctctggatccactgcttaaatacggacgaggacagggccctgtctcctcagcttcaggcaccaccactgacctgggacagtgaatcgacaatgccgtcttctgtctcgtggggcatcctcctgctggcaggcctgtgctgcctggtccctgtctccctggctgaggatccccagggagatgctgcccagaagacagatacatcccaccatgatcaggatcacccaaccttcaacaagatcacccccaacctggctgagttcgccttcagcctataccgccagctggcacaccagtccaacagcaccaatatcttcttctccccagtgagcatcgctacagcctttgcaatgctctccctggggaccaaggctgacactcacgatgaaatcctggagggcctgaatttcaacctcacggagattccggaggctcagatccatgaaggcttccaggaactcctccgtaccctcaaccagccagacagccagctccagctgaccaccggcaatggcctgttcctcagcgagggcctgaagctagtggataagtttttggaggatgttaaaaagttgtaccactcagaagccttcactgtcaacttcggggacaccgaagaggccaagaaacagatcaacgattacgtggagaagggtactcaagggaaaattgtggatttggtcaaggagcttgacagagacacagtttttgctctggtgaattacatcttctttaaaggcaaatgggagagaccctttgaagtcaaggacaccgaggaagaggacttccacgtggaccaggtgaccaccgtgaaggtgcctatgatgaagcgtttaggcatgtttaacatccagcactgtaagaagctgtccagctgggtgctgctgatgaaatacctgggcaatgccaccgccatcttcttcctgcctgatgaggggaaactacagcacctggaaaatgaactcacccacgatatcatcaccaagttcctggaaaatgaagacagaaggtctgccagcttacatttacccaaactgtccattactggaacctatgatctgaagagcgtcctgggtcaactgggcatcactaaggtcttcagcaatggggctgacctctccggggtcacagaggaggcacccctgaagctctccaaggccgtgcataaggctgtgctgaccatcgacgagaaagggactgaagctgctggggccatgtttttagaggccatacccatgtctatcccccccgaggtcaagttcaacaaaccctttgtcttcttaatgattgaacaaaataccaagtctcccctcttcatgggaaaagtggtgaatcccacccaaaaataactgcctctcgctcctcaacccctcccctccatccctggccccctccctggatgacattaaagaagggttgagctggtccctgcctgcatgtgactgtaaatccctcccatgttttctctgagtctccctttgcctgctgaggctgtatgtgggctccaggtaacagtgctgtcttcgggccccctgaactgtgttcatggagcatctggctgggtaggcacatgctgggcttgaatccaggggggactgaatcctcagcttacggacctgggcccatctgtttctggagggctccagtcttccttgtcctgtcttggagtccccaagaaggaatcacaggggaggaaccagataccagccatgaccccaggctccaccaagcatcttcatgtccccctgctcatcccccactcccccccacccagagttgctcatcctgccagggctggctgtgcccaccccaaggctgccctcctgggggccccagaactgcctgatcgtgccgtggcccagttttgtggcatctgcagcaacacaagagagaggacaatgtcctcctcttgacccgctgtcacctaaccagactcgggccctgcacctctcaggcacttctggaaaatgactgaggcagattcttcctgaagcccattctccatggggcaacaaggacacctattctgtccttgtccttccatcgctgccccagaaagcctcacatatctccgtttagaatcaggtcccttctccccagatgaagaggagggtctctgctttgttttctctatctcctcctcagacttgaccaggcccagcaggccccagaagaccattaccctatatcccttctcctccctagtcacatggccataggcctgctgatggctcaggaaggccattgcaaggactcctcagctatgggagaggaagcacatcacccattgacccccgcaacccctccctttcctcctctgagtcccgactggggccacatgcagcctgacttctttgtgcctgttgctgtccctgcagtcttcagagggccaccgcagctccagtgccacggcaggaggctgttcctgaatagcccctgtggtaagggccaggagagtccttccatcctccaaggccctgctaaaggacacagcagccaggaagtcccctgggcccctagctgaaggacagcctgctccctccgtctctaccaggaatggccttgtcctatggaaggcactgccccatcccaaactaatctaggaatcactgtctaaccactcactgtcatgaatgtgtacttaaaggatgaggttgagtcataccaaatagtgatttcgatagttcaaaatggtgaaattagcaattctacatgattcagtctaatcaatggataccgactgtttcccacacaagtctcctgttctcttaagcttactcactgacagcctttcactctccacaaatacattaaagatatggccatcaccaagccccctaggatgacaccagacctgagagtctgaagacctggatccaagttctgacttttccccctgacagctgtgtgaccttcgtgaagtcgccaaacctctctgagccccagtcattgctagtaagacctgcctttgagttggtatgatgttcaagttagataacaaaatgtttatacccattagaacagagaataaatagaactacatttcttgca

SEQ ID NO: 10 - DNA, 3303 bp, Homo sapiens
tgggcaggaactgggcactgtgcccagggcatgcactgcctccacgcagcaaccctcagagtcctgagctgaaccaagaaggaggagggggtcgggcctccgaggaaggcctagccgctgctgctgccaggaattccaggttggaggggcggcaacctcctgccagccttcaggccactctcctgtgcctgccagaagagacagagcttgaggagagcttgaggagagcaggaaagcagcctcccccgttgcccctctggatccactgcttaaatacggacgaggacagggccctgtctcctcagcttcaggcaccaccactgacctgggacagtgaatcgacaatgccgtcttctgtctcgtggggcatcctcctgctggcaggcctgtgctgcctggtccctgtctccctggctgaggatccccagggagatgctgcccagaagacagatacatcccaccatgatcaggatcacccaaccttcaacaagatcacccccaacctggctgagttcgccttcagcctataccgccagctggcacaccagtccaacagcaccaatatcttcttctccccagtgagcatcgctacagcctttgcaatgctctccctggggaccaaggctgacactcacgatgaaatcctggagggcctgaatttcaacctcacggagattccggaggctcagatccatgaaggcttccaggaactcctccgtaccctcaaccagccagacagccagctccagctgaccaccggcaatggcctgttcctcagcgagggcctgaagctagtggataagtttttggaggatgttaaaaagttgtaccactcagaagccttcactgtcaacttcggggacaccgaagaggccaagaaacagatcaacgattacgtggagaagggtactcaagggaaaattgtggatttggtcaaggagcttgacagagacacagtttttgctctggtgaattacatcttctttaaaggcaaatgggagagaccctttgaagtcaaggacaccgaggaagaggacttccacgtggaccaggtgaccaccgtgaaggtgcctatgatgaagcgtttaggcatgtttaacatccagcactgtaagaagctgtccagctgggtgctgctgatgaaatacctgggcaatgccaccgccatcttcttcctgcctgatgaggggaaactacagcacctggaaaatgaactcacccacgatatcatcaccaagttcctggaaaatgaagacagaaggtctgccagcttacatttacccaaactgtccattactggaacctatgatctgaagagcgtcctgggtcaactgggcatcactaaggtcttcagcaatggggctgacctctccggggtcacagaggaggcacccctgaagctctccaaggccgtgcataaggctgtgctgaccatcgacgagaaagggactgaagctgctggggccatgtttttagaggccatacccatgtctatcccccccgaggtcaagttcaacaaaccctttgtcttcttaatgattgaacaaaataccaagtctcccctcttcatgggaaaagtggtgaatcccacccaaaaataactgcctctcgctcctcaacccctcccctccatccctggccccctccctggatgacattaaagaagggttgagctggtccctgcctgcatgtgactgtaaatccctcccatgttttctctgagtctccctttgcctgctgaggctgtatgtgggctccaggtaacagtgctgtcttcgggccccctgaactgtgttcatggagcatctggctgggtaggcacatgctgggcttgaatccaggggggactgaatcctcagcttacggacctgggcccatctgtttctggagggctccagtcttccttgtcctgtcttggagtccccaagaaggaatcacaggggaggaaccagataccagccatgaccccaggctccaccaagcatcttcatgtccccctgctcatcccccactcccccccacccagagttgctcatcctgccagggctggctgtgcccaccccaaggctgccctcctgggggccccagaactgcctgatcgtgccgtggcccagttttgtggcatctgcagcaacacaagagagaggacaatgtcctcctcttgacccgctgtcacctaaccagactcgggccctgcacctctcaggcacttctggaaaatgactgaggcagattcttcctgaagcccattctccatggggcaacaaggacacctattctgtccttgtccttccatcgctgccccagaaagcctcacatatctccgtttagaatcaggtcccttctccccagatgaagaggagggtctctgctttgttttctctatctcctcctcagacttgaccaggcccagcaggccccagaagaccattaccctatatcccttctcctccctagtcacatggccataggcctgctgatggctcaggaaggccattgcaaggactcctcagctatgggagaggaagcacatcacccattgacccccgcaacccctccctttcctcctctgagtcccgactggggccacatgcagcctgacttctttgtgcctgttgctgtccctgcagtcttcagagggccaccgcagctccagtgccacggcaggaggctgttcctgaatagcccctgtggtaagggccaggagagtccttccatcctccaaggccctgctaaaggacacagcagccaggaagtcccctgggcccctagctgaaggacagcctgctccctccgtctctaccaggaatggccttgtcctatggaaggcactgccccatcccaaactaatctaggaatcactgtctaaccactcactgtcatgaatgtgtacttaaaggatgaggttgagtcataccaaatagtgatttcgatagttcaaaatggtgaaattagcaattctacatgattcagtctaatcaatggataccgactgtttcccacacaagtctcctgttctcttaagcttactcactgacagcctttcactctccacaaatacattaaagatatggccatcaccaagccccctaggatgacaccagacctgagagtctgaagacctggatccaagttctgacttttccccctgacagctgtgtgaccttcgtgaagtcgccaaacctctctgagccccagtcattgctagtaagacctgcctttgagttggtatgatgttcaagttagataacaaaatgtttatacccattagaacagagaataaatagaactacatttcttgca

SEQ ID NO: 11 - DNA, 3300 bp, Homo sapiens
tgggcaggaactgggcactgtgcccagggcatgcactgcctccacgcagcaaccctcagagtcctgagctgaaccaagaaggaggagggggtcgggcctccgaggaaggcctagccgctgctgctgccaggaattccaggttggaggggcggcaacctcctgccagccttcaggccactctcctgtgcctgccagaagagacagagcttgaggagagcttgaggagagcaggaaagcctcccccgttgcccctctggatccactgcttaaatacggacgaggacagggccctgtctcctcagcttcaggcaccaccactgacctgggacagtgaatcgacaatgccgtcttctgtctcgtggggcatcctcctgctggcaggcctgtgctgcctggtccctgtctccctggctgaggatccccagggagatgctgcccagaagacagatacatcccaccatgatcaggatcacccaaccttcaacaagatcacccccaacctggctgagttcgccttcagcctataccgccagctggcacaccagtccaacagcaccaatatcttcttctccccagtgagcatcgctacagcctttgcaatgctctccctggggaccaaggctgacactcacgatgaaatcctggagggcctgaatttcaacctcacggagattccggaggctcagatccatgaaggcttccaggaactcctccgtaccctcaaccagccagacagccagctccagctgaccaccggcaatggcctgttcctcagcgagggcctgaagctagtggataagtttttggaggatgttaaaaagttgtaccactcagaagccttcactgtcaacttcggggacaccgaagaggccaagaaacagatcaacgattacgtggagaagggtactcaagggaaaattgtggatttggtcaaggagcttgacagagacacagtttttgctctggtgaattacatcttctttaaaggcaaatgggagagaccctttgaagtcaaggacaccgaggaagaggacttccacgtggaccaggtgaccaccgtgaaggtgcctatgatgaagcgtttaggcatgtttaacatccagcactgtaagaagctgtccagctgggtgctgctgatgaaatacctgggcaatgccaccgccatcttcttcctgcctgatgaggggaaactacagcacctggaaaatgaactcacccacgatatcatcaccaagttcctggaaaatgaagacagaaggtctgccagcttacatttacccaaactgtccattactggaacctatgatctgaagagcgtcctgggtcaactgggcatcactaaggtcttcagcaatggggctgacctctccggggtcacagaggaggcacccctgaagctctccaaggccgtgcataaggctgtgctgaccatcgacgagaaagggactgaagctgctggggccatgtttttagaggccatacccatgtctatcccccccgaggtcaagttcaacaaaccctttgtcttcttaatgattgaacaaaataccaagtctcccctcttcatgggaaaagtggtgaatcccacccaaaaataactgcctctcgctcctcaacccctcccctccatccctggccccctccctggatgacattaaagaagggttgagctggtccctgcctgcatgtgactgtaaatccctcccatgttttctctgagtctccctttgcctgctgaggctgtatgtgggctccaggtaacagtgctgtcttcgggccccctgaactgtgttcatggagcatctggctgggtaggcacatgctgggcttgaatccaggggggactgaatcctcagcttacggacctgggcccatctgtttctggagggctccagtcttccttgtcctgtcttggagtccccaagaaggaatcacaggggaggaaccagataccagccatgaccccaggctccaccaagcatcttcatgtccccctgctcatcccccactcccccccacccagagttgctcatcctgccagggctggctgtgcccaccccaaggctgccctcctgggggccccagaactgcctgatcgtgccgtggcccagttttgtggcatctgcagcaacacaagagagaggacaatgtcctcctcttgacccgctgtcacctaaccagactcgggccctgcacctctcaggcacttctggaaaatgactgaggcagattcttcctgaagcccattctccatggggcaacaaggacacctattctgtccttgtccttccatcgctgccccagaaagcctcacatatctccgtttagaatcaggtcccttctccccagatgaagaggagggtctctgctttgttttctctatctcctcctcagacttgaccaggcccagcaggccccagaagaccattaccctatatcccttctcctccctagtcacatggccataggcctgctgatggctcaggaaggccattgcaaggactcctcagctatgggagaggaagcacatcacccattgacccccgcaacccctccctttcctcctctgagtcccgactggggccacatgcagcctgacttctttgtgcctgttgctgtccctgcagtcttcagagggccaccgcagctccagtgccacggcaggaggctgttcctgaatagcccctgtggtaagggccaggagagtccttccatcctccaaggccctgctaaaggacacagcagccaggaagtcccctgggcccctagctgaaggacagcctgctccctccgtctctaccaggaatggccttgtcctatggaaggcactgccccatcccaaactaatctaggaatcactgtctaaccactcactgtcatgaatgtgtacttaaaggatgaggttgagtcataccaaatagtgatttcgatagttcaaaatggtgaaattagcaattctacatgattcagtctaatcaatggataccgactgtttcccacacaagtctcctgttctcttaagcttactcactgacagcctttcactctccacaaatacattaaagatatggccatcaccaagccccctaggatgacaccagacctgagagtctgaagacctggatccaagttctgacttttccccctgacagctgtgtgaccttcgtgaagtcgccaaacctctctgagccccagtcattgctagtaagacctgcctttgagttggtatgatgttcaagttagataacaaaatgtttatacccattagaacagagaataaatagaactacatttcttgca

SEQ ID NO: 12 - DNA, 2064 bp, Macaca mulatta
gcccagtcttgtgtctgcctggcaatgggcaaggccccttcctgcccaagctccccgcccctccccaacctattgcctccgccacccgccacccgaggccaacttcctgggtgggcaggaactgggccctgtgcccagggcgtgcactgcctccacgcagcaaccctcagagtactgagctgagcaaaggaggaggaggggatcagcactctgaggaaggcctagccactgctgctgccaggaattccagggcggcatcagtcttcagcatcaggcatttcggggtgaattagtaaatggtagatcttgctaccagtggaacagccgctaaggattctgcagtgagagcagagggccagcaaagtggtactctcccagcgactggctgactcacgccaccccctccaccttggacgcaggacactgtggtttctgagccaggtacaatgactccttttggtacgtgcagtggaggctgtatgctgctcaggcagagcgtccggacagcgtgggcgggcgactcagcgcccagcctgtgaacttagtccctgtttgctcctccggtaactggggtgatcttggttaatattcaccagcagcctcccccgttgcccctctgcacccactgcttaaatacggacaaggacagggctctgtctcctcagcctcaggcaccaccactgacctgggacggtgaatcgacaatgccatcttctgtctcatggggcgtcctcctgctggcaggcctgtgctgcctgctccccggctctctggctgaggatccccagggagatgctgcccagaagacggatacatcccaccatgatcaggaccacccaaccctcaacaagatcacccccagcctggctgagttcggcttcagcctataccgccagctggcacaccagtccaacagcaccaatatcttcttctccccagtgagcatcgctacagcctttgcaatgctctccctggggaccaaggctgacactcacagtgaaatcctggagggcctgaatttcaacgtcacggagattccggaggctcaggtccatgaaggcttccaggaactcctccataccctcaacaagccagacagccagctccagctgaccaccggcaacggcctgttcctcaacaagagcctgaaggtagtggataagtttttggaggatgtcaaaaaactgtaccactcagaagccttctctgtcaactttgaggacaccgaagaggccaagaaacagatcaacaattacgtggagaaggaaactcaagggaaaattgtggatttggtcaaggagcttgacagagacacagtttttgctctggtgaattacatcttctttaaaggcaaatgggagagaccctttgacgttgaggccaccaaggaagaggacttccacgtggaccaggcgaccaccgtgaaggtgcccatgatgaggcgtttaggcatgtttaacatctaccactgtgagaagctgtccagctgggtgctgctgatgaaatacctgggcaatgccaccgccatcttcttcctgcctgatgaggggaaactgcagcacctggaaaatgaactcacccatgatatcatcaccaagttcctggaaaatgaaaacagcaggtctgccaacttacatttacccagactggccattactggaacctatgatctgaagacagtcctgggccacctgggtatcactaaggtcttcagcaatggggctgacctctcggggatcacggaggaggcacccctgaagctctccaaggccgtgcataaggctgtgctgaccatcgatgagaaagggactgaagctgctggggccatgtttttagaggccatacccatgtctattccccccgaggtcaagttcaacaaaccctttgtcttcttaatgattgaacaaaataccaagtctcccctcttcatgggaaaagtggtgaatcccacccagaaataactgcctgtcactcctcagcccctcccctccatccctggccccctccctgaatgacattaaagaagggttgagctggtccctgcctgcgtgtgtgactgcaaac

SEQ ID NO: 13 - DNA, 1608 bp, Macaca mulatta
tcttgtgtctgcctggcaatgggcaaggccccttcctgcccaagctccccgcccctccccaacctattgcctccgccacccgccacccgaggccaacttcctgggtgggcaggaactgggccctgtgcccagggcgtgcactgcctccacgcagcaaccctcagagtactgagctgagcaaaggaggaggaggggatcagcactctgaggaaggcctagccactgctgctgccaggaattccaggacaatgccatcttctgtctcatggggcgtcctcctgctggcaggcctgtgctgcctgctccccggctctctggctgaggatccccagggagatgctgcccagaagacggatacatcccaccatgatcaggaccacccaaccctcaacaagatcacccccagcctggctgagttcggcttcagcctataccgccagctggcacaccagtccaacagcaccaatatcttcttctccccagtgagcatcgctacagcctttgcaatgctctccctggggaccaaggctgacactcacagtgaaatcctggagggcctgaatttcaacgtcacggagattccggaggctcaggtccatgaaggcttccaggaactcctccataccctcaacaagccagacagccagctccagctgaccaccggcaacggcctgttcctcaacaagagcctgaaggtagtggataagtttttggaggatgtcaaaaaactgtaccactcagaagccttctctgtcaactttgaggacaccgaagaggccaagaaacagatcaacaattacgtggagaaggaaactcaagggaaaattgtggatttggtcaaggagcttgacagagacacagtttttgctctggtgaattacatcttctttaaaggcaaatgggagagaccctttgacgttgaggccaccaaggaagaggacttccacgtggaccaggcgaccaccgtgaaggtgcccatgatgaggcgtttaggcatgtttaacatctaccactgtgagaagctgtccagctgggtgctgctgatgaaatacctgggcaatgccaccgccatcttcttcctgcctgatgaggggaaactgcagcacctggaaaatgaactcacccatgatatcatcaccaagttcctggaaaatgaaaacagcaggtctgccaacttacatttacccagactggccattactggaacctatgatctgaagacagtcctgggccacctgggtatcactaaggtcttcagcaatggggctgacctctcggggatcacggaggaggcacccctgaagctctccaaggccgtgcataaggctgtgctgaccatcgatgagaaagggactgaagctgctggggccatgtttttagaggccatacccatgtctattccccccgaggtcaagttcaacaaaccctttgtcttcttaatgattgaacaaaataccaagtctcccctcttcatgggaaaagtggtgaatcccacccagaaataactgcctgtcactcctcagcccctcccctccatccctggccccctccctgaatgacattaaagaagggttgagctggtccctgcctgcgtgtgtgactgcaaac

SEQ ID NO: 14 - DNA, 3220 bp, Homo sapiens
tgcaagaaatgtagttctatttattctctgttctaatgggtataaacattttgttatctaacttgaacatcataccaactcaaaggcaggtcttactagcaatgactggggctcagagaggtttggcgacttcacgaaggtcacacagctgtcagggggaaaagtcagaacttggatccaggtcttcagactctcaggtctggtgtcatcctagggggcttggtgatggccatatctttaatgtatttgtggagagtgaaaggctgtcagtgagtaagcttaagagaacaggagacttgtgtgggaaacagtcggtatccattgattagactgaatcatgtagaattgctaatttcaccattttgaactatcgaaatcactatttggtatgactcaacctcatcctttaagtacacattcatgacagtgagtggttagacagtgattcctagattagtttgggatggggcagtgccttccataggacaaggccattcctggtagagacggagggagcaggctgtccttcagctaggggcccaggggacttcctggctgctgtgtcctttagcagggccttggaggatggaaggactctcctggcccttaccacaggggctattcaggaacagcctcctgccgtggcactggagctgcggtggccctctgaagactgcagggacagcaacaggcacaaagaagtcaggctgcatgtggccccagtcgggactcagaggaggaaagggaggggttgcgggggtcaatgggtgatgtgcttcctctcccatagctgaggagtccttgcaatggccttcctgagccatcagcaggcctatggccatgtgactagggaggagaagggatatagggtaatggtcttctggggcctgctgggcctggtcaagtctgaggaggagatagagaaaacaaagcagagaccctcctcttcatctggggagaagggacctgattctaaacggagatatgtgaggctttctggggcagcgatggaaggacaaggacagaataggtgtccttgttgccccatggagaatgggcttcaggaagaatctgcctcagtcattttccagaagtgcctgagaggtgcagggcccgagtctggttaggtgacagcgggtcaagaggaggacattgtcctctctcttgtgttgctgcagatgccacaaaactgggccacggcacgatcaggcagttctggggcccccaggagggcagccttggggtgggcacagccagccctggcaggatgagcaactctgggtgggggggagtgggggatgagcagggggacatgaagatgcttggtggagcctggggtcatggctggtatctggttcctcccctgtgattccttcttggggactccaagacaggacaaggaagactggagccctccagaaacagatgggcccaggtccgtaagctgaggattcagtcccccctggattcaagcccagcatgtgcctacccagccagatgctccatgaacacagttcagggggcccgaagacagcactgttacctggagcccacatacagcctcagcaggcaaagggagactcagagaaaacatgggagggatttacagtcacatgcaggcagggaccagctcaacccttctttaatgtcatccagggagggggccagggatggaggggaggggttgaggagcgagaggcagttatttttgggtgggattcaccacttttcccatgaagaggggagacttggtattttgttcaatcattaagaagacaaagggtttgttgaacttgacctcgggggggatagacatgggtatggcctctaaaaacatggccccagcagcttcagtccctttctcgtcgatggtcagcacagccttatgcacggccttggagagcttcaggggtgcctcctctgtgaccccggagaggtcagccccattgctgaagaccttagtgatgcccagttgacccaggacgctcttcagatcataggttccagtaatggacagtttgggtaaatgtaagctggcagaccttctgtcttcattttccaggaacttggtgatgatatcgtgggtgagttcattttccaggtgctgtagtttcccctcatcaggcaggaagaagatggcggtggcattgcccaggtatttcatcagcagcacccagctggacagcttcttacagtgctggatgttaaacatgcctaaacgcttcatcataggcaccttcacggtggtcacctggtccacgtggaagtcctcttcctcggtgtccttgacttcaaagggtctctcccatttgcctttaaagaagatgtaattcaccagagcaaaaactgtgtctctgtcaagctccttgaccaaatccacaattttcccttgagtacccttctccacgtaatcgttgatctgtttcttggcctcttcggtgtccccgaagttgacagtgaaggcttctgagtggtacaactttttaacatcctccaaaaacttatccactagcttcaggccctcgctgaggaacaggccattgccggtggtcagctggagctggctgtctggctggttgagggtacggaggagttcctggaagccttcatggatctgagcctccggaatctccgtgaggttgaaattcaggccctccaggatttcatcgtgagtgtcagccttggtccccagggagagcattgcaaaggctgtagcgatgctcactggggagaagaagatattggtgctgttggactggtgtgccagctggcggtataggctgaaggcgaactcagccaggttgggggtgatcttgttgaaggttgggtgatcctgatcatggtgggatgtatctgtcttctgggcagcatctccctggggatcctcagccagggagacagggaccaggcagcacaggcctgccagcaggaggatgccccacgagacagaagacggcattgtcgattcactgtcccaggtcagtggtggtgcctgaagctgaggagacagggccctgtcctcgtccgtatttaagcagtggatccagaggggcaacgggggaggctgctggtgaatattaaccaaggtcaccccagttatcggaggagcaaacaggggctaagtccactggctgggatctgagtcgcccgcctacgctgcccggacgctttgcctgggcagtgtacagcttccactgcacttaccgaaaggagtcattgt

SEQ ID NO: 15 - DNA, 3199 bp, Homo sapiens
tgcaagaaatgtagttctatttattctctgttctaatgggtataaacattttgttatctaacttgaacatcataccaactcaaaggcaggtcttactagcaatgactggggctcagagaggtttggcgacttcacgaaggtcacacagctgtcagggggaaaagtcagaacttggatccaggtcttcagactctcaggtctggtgtcatcctagggggcttggtgatggccatatctttaatgtatttgtggagagtgaaaggctgtcagtgagtaagcttaagagaacaggagacttgtgtgggaaacagtcggtatccattgattagactgaatcatgtagaattgctaatttcaccattttgaactatcgaaatcactatttggtatgactcaacctcatcctttaagtacacattcatgacagtgagtggttagacagtgattcctagattagtttgggatggggcagtgccttccataggacaaggccattcctggtagagacggagggagcaggctgtccttcagctaggggcccaggggacttcctggctgctgtgtcctttagcagggccttggaggatggaaggactctcctggcccttaccacaggggctattcaggaacagcctcctgccgtggcactggagctgcggtggccctctgaagactgcagggacagcaacaggcacaaagaagtcaggctgcatgtggccccagtcgggactcagaggaggaaagggaggggttgcgggggtcaatgggtgatgtgcttcctctcccatagctgaggagtccttgcaatggccttcctgagccatcagcaggcctatggccatgtgactagggaggagaagggatatagggtaatggtcttctggggcctgctgggcctggtcaagtctgaggaggagatagagaaaacaaagcagagaccctcctcttcatctggggagaagggacctgattctaaacggagatatgtgaggctttctggggcagcgatggaaggacaaggacagaataggtgtccttgttgccccatggagaatgggcttcaggaagaatctgcctcagtcattttccagaagtgcctgagaggtgcagggcccgagtctggttaggtgacagcgggtcaagaggaggacattgtcctctctcttgtgttgctgcagatgccacaaaactgggccacggcacgatcaggcagttctggggcccccaggagggcagccttggggtgggcacagccagccctggcaggatgagcaactctgggtgggggggagtgggggatgagcagggggacatgaagatgcttggtggagcctggggtcatggctggtatctggttcctcccctgtgattccttcttggggactccaagacaggacaaggaagactggagccctccagaaacagatgggcccaggtccgtaagctgaggattcagtcccccctggattcaagcccagcatgtgcctacccagccagatgctccatgaacacagttcagggggcccgaagacagcactgttacctggagcccacatacagcctcagcaggcaaagggagactcagagaaaacatgggagggatttacagtcacatgcaggcagggaccagctcaacccttctttaatgtcatccagggagggggccagggatggaggggaggggttgaggagcgagaggcagttatttttgggtgggattcaccacttttcccatgaagaggggagacttggtattttgttcaatcattaagaagacaaagggtttgttgaacttgacctcgggggggatagacatgggtatggcctctaaaaacatggccccagcagcttcagtccctttctcgtcgatggtcagcacagccttatgcacggccttggagagcttcaggggtgcctcctctgtgaccccggagaggtcagccccattgctgaagaccttagtgatgcccagttgacccaggacgctcttcagatcataggttccagtaatggacagtttgggtaaatgtaagctggcagaccttctgtcttcattttccaggaacttggtgatgatatcgtgggtgagttcattttccaggtgctgtagtttcccctcatcaggcaggaagaagatggcggtggcattgcccaggtatttcatcagcagcacccagctggacagcttcttacagtgctggatgttaaacatgcctaaacgcttcatcataggcaccttcacggtggtcacctggtccacgtggaagtcctcttcctcggtgtccttgacttcaaagggtctctcccatttgcctttaaagaagatgtaattcaccagagcaaaaactgtgtctctgtcaagctccttgaccaaatccacaattttcccttgagtacccttctccacgtaatcgttgatctgtttcttggcctcttcggtgtccccgaagttgacagtgaaggcttctgagtggtacaactttttaacatcctccaaaaacttatccactagcttcaggccctcgctgaggaacaggccattgccggtggtcagctggagctggctgtctggctggttgagggtacggaggagttcctggaagccttcatggatctgagcctccggaatctccgtgaggttgaaattcaggccctccaggatttcatcgtgagtgtcagccttggtccccagggagagcattgcaaaggctgtagcgatgctcactggggagaagaagatattggtgctgttggactggtgtgccagctggcggtataggctgaaggcgaactcagccaggttgggggtgatcttgttgaaggttgggtgatcctgatcatggtgggatgtatctgtcttctgggcagcatctccctggggatcctcagccagggagacagggaccaggcagcacaggcctgccagcaggaggatgccccacgagacagaagacggcattgtcctttcctgctctcctcaagctctcctcaagctctgtctcttctggcaggcacaggagagtggcctgaaggctggcaggaggttgccgcccctccaacctggaattcctggcagcagcagcggctaggccttcctcggaggcccgaccccctcctccttcttggttcagctcaggactctgagggttgctgcgtggaggcagtgcatgccctgggcacagtgcccagttcctgccca

SEQ ID NO: 16 - DNA, 3513 bp, Homo sapiens
tgcaagaaatgtagttctatttattctctgttctaatgggtataaacattttgttatctaacttgaacatcataccaactcaaaggcaggtcttactagcaatgactggggctcagagaggtttggcgacttcacgaaggtcacacagctgtcagggggaaaagtcagaacttggatccaggtcttcagactctcaggtctggtgtcatcctagggggcttggtgatggccatatctttaatgtatttgtggagagtgaaaggctgtcagtgagtaagcttaagagaacaggagacttgtgtgggaaacagtcggtatccattgattagactgaatcatgtagaattgctaatttcaccattttgaactatcgaaatcactatttggtatgactcaacctcatcctttaagtacacattcatgacagtgagtggttagacagtgattcctagattagtttgggatggggcagtgccttccataggacaaggccattcctggtagagacggagggagcaggctgtccttcagctaggggcccaggggacttcctggctgctgtgtcctttagcagggccttggaggatggaaggactctcctggcccttaccacaggggctattcaggaacagcctcctgccgtggcactggagctgcggtggccctctgaagactgcagggacagcaacaggcacaaagaagtcaggctgcatgtggccccagtcgggactcagaggaggaaagggaggggttgcgggggtcaatgggtgatgtgcttcctctcccatagctgaggagtccttgcaatggccttcctgagccatcagcaggcctatggccatgtgactagggaggagaagggatatagggtaatggtcttctggggcctgctgggcctggtcaagtctgaggaggagatagagaaaacaaagcagagaccctcctcttcatctggggagaagggacctgattctaaacggagatatgtgaggctttctggggcagcgatggaaggacaaggacagaataggtgtccttgttgccccatggagaatgggcttcaggaagaatctgcctcagtcattttccagaagtgcctgagaggtgcagggcccgagtctggttaggtgacagcgggtcaagaggaggacattgtcctctctcttgtgttgctgcagatgccacaaaactgggccacggcacgatcaggcagttctggggcccccaggagggcagccttggggtgggcacagccagccctggcaggatgagcaactctgggtgggggggagtgggggatgagcagggggacatgaagatgcttggtggagcctggggtcatggctggtatctggttcctcccctgtgattccttcttggggactccaagacaggacaaggaagactggagccctccagaaacagatgggcccaggtccgtaagctgaggattcagtcccccctggattcaagcccagcatgtgcctacccagccagatgctccatgaacacagttcagggggcccgaagacagcactgttacctggagcccacatacagcctcagcaggcaaagggagactcagagaaaacatgggagggatttacagtcacatgcaggcagggaccagctcaacccttctttaatgtcatccagggagggggccagggatggaggggaggggttgaggagcgagaggcagttatttttgggtgggattcaccacttttcccatgaagaggggagacttggtattttgttcaatcattaagaagacaaagggtttgttgaacttgacctcgggggggatagacatgggtatggcctctaaaaacatggccccagcagcttcagtccctttctcgtcgatggtcagcacagccttatgcacggccttggagagcttcaggggtgcctcctctgtgaccccggagaggtcagccccattgctgaagaccttagtgatgcccagttgacccaggacgctcttcagatcataggttccagtaatggacagtttgggtaaatgtaagctggcagaccttctgtcttcattttccaggaacttggtgatgatatcgtgggtgagttcattttccaggtgctgtagtttcccctcatcaggcaggaagaagatggcggtggcattgcccaggtatttcatcagcagcacccagctggacagcttcttacagtgctggatgttaaacatgcctaaacgcttcatcataggcaccttcacggtggtcacctggtccacgtggaagtcctcttcctcggtgtccttgacttcaaagggtctctcccatttgcctttaaagaagatgtaattcaccagagcaaaaactgtgtctctgtcaagctccttgaccaaatccacaattttcccttgagtacccttctccacgtaatcgttgatctgtttcttggcctcttcggtgtccccgaagttgacagtgaaggcttctgagtggtacaactttttaacatcctccaaaaacttatccactagcttcaggccctcgctgaggaacaggccattgccggtggtcagctggagctggctgtctggctggttgagggtacggaggagttcctggaagccttcatggatctgagcctccggaatctccgtgaggttgaaattcaggccctccaggatttcatcgtgagtgtcagccttggtccccagggagagcattgcaaaggctgtagcgatgctcactggggagaagaagatattggtgctgttggactggtgtgccagctggcggtataggctgaaggcgaactcagccaggttgggggtgatcttgttgaaggttgggtgatcctgatcatggtgggatgtatctgtcttctgggcagcatctccctggggatcctcagccagggagacagggaccaggcagcacaggcctgccagcaggaggatgccccacgagacagaagacggcattgtcgattcactgtcccaggtcagtggtggtgcctgaagctgaggagacagggccctgtcctcgtccgtatttaagcagtggatccagaggggcaacgggggaggctgcgaaaggagtcattgtacctggctcagaaaccacagcgtcctgtgtccaaggtggagggggtggcgtgagtcagacagtctctgggagagtaccacttagctggccctctgctctcactgcagaatccttagtggctgttccactggtagcaagatctaccatttactgagtcaccccaaaatgcctgatgctgaagacttactgccgccctttcctgctctcctcaagctctcctcaagctctgtctcttctggcaggcacaggagagtggcctgaaggctggcaggaggttgccgcccctccaacctggaattcctggcagcagcagcggctaggccttcctcggaggcccgaccccctcctccttcttggttcagctcaggactctgagggttgctgcgtggaggcagtgcatgccctgggcacagtgcccagttcctgccca

SEQ ID NO: 17 - DNA, 3236 bp, Homo sapiens
tgcaagaaatgtagttctatttattctctgttctaatgggtataaacattttgttatctaacttgaacatcataccaactcaaaggcaggtcttactagcaatgactggggctcagagaggtttggcgacttcacgaaggtcacacagctgtcagggggaaaagtcagaacttggatccaggtcttcagactctcaggtctggtgtcatcctagggggcttggtgatggccatatctttaatgtatttgtggagagtgaaaggctgtcagtgagtaagcttaagagaacaggagacttgtgtgggaaacagtcggtatccattgattagactgaatcatgtagaattgctaatttcaccattttgaactatcgaaatcactatttggtatgactcaacctcatcctttaagtacacattcatgacagtgagtggttagacagtgattcctagattagtttgggatggggcagtgccttccataggacaaggccattcctggtagagacggagggagcaggctgtccttcagctaggggcccaggggacttcctggctgctgtgtcctttagcagggccttggaggatggaaggactctcctggcccttaccacaggggctattcaggaacagcctcctgccgtggcactggagctgcggtggccctctgaagactgcagggacagcaacaggcacaaagaagtcaggctgcatgtggccccagtcgggactcagaggaggaaagggaggggttgcgggggtcaatgggtgatgtgcttcctctcccatagctgaggagtccttgcaatggccttcctgagccatcagcaggcctatggccatgtgactagggaggagaagggatatagggtaatggtcttctggggcctgctgggcctggtcaagtctgaggaggagatagagaaaacaaagcagagaccctcctcttcatctggggagaagggacctgattctaaacggagatatgtgaggctttctggggcagcgatggaaggacaaggacagaataggtgtccttgttgccccatggagaatgggcttcaggaagaatctgcctcagtcattttccagaagtgcctgagaggtgcagggcccgagtctggttaggtgacagcgggtcaagaggaggacattgtcctctctcttgtgttgctgcagatgccacaaaactgggccacggcacgatcaggcagttctggggcccccaggagggcagccttggggtgggcacagccagccctggcaggatgagcaactctgggtgggggggagtgggggatgagcagggggacatgaagatgcttggtggagcctggggtcatggctggtatctggttcctcccctgtgattccttcttggggactccaagacaggacaaggaagactggagccctccagaaacagatgggcccaggtccgtaagctgaggattcagtcccccctggattcaagcccagcatgtgcctacccagccagatgctccatgaacacagttcagggggcccgaagacagcactgttacctggagcccacatacagcctcagcaggcaaagggagactcagagaaaacatgggagggatttacagtcacatgcaggcagggaccagctcaacccttctttaatgtcatccagggagggggccagggatggaggggaggggttgaggagcgagaggcagttatttttgggtgggattcaccacttttcccatgaagaggggagacttggtattttgttcaatcattaagaagacaaagggtttgttgaacttgacctcgggggggatagacatgggtatggcctctaaaaacatggccccagcagcttcagtccctttctcgtcgatggtcagcacagccttatgcacggccttggagagcttcaggggtgcctcctctgtgaccccggagaggtcagccccattgctgaagaccttagtgatgcccagttgacccaggacgctcttcagatcataggttccagtaatggacagtttgggtaaatgtaagctggcagaccttctgtcttcattttccaggaacttggtgatgatatcgtgggtgagttcattttccaggtgctgtagtttcccctcatcaggcaggaagaagatggcggtggcattgcccaggtatttcatcagcagcacccagctggacagcttcttacagtgctggatgttaaacatgcctaaacgcttcatcataggcaccttcacggtggtcacctggtccacgtggaagtcctcttcctcggtgtccttgacttcaaagggtctctcccatttgcctttaaagaagatgtaattcaccagagcaaaaactgtgtctctgtcaagctccttgaccaaatccacaattttcccttgagtacccttctccacgtaatcgttgatctgtttcttggcctcttcggtgtccccgaagttgacagtgaaggcttctgagtggtacaactttttaacatcctccaaaaacttatccactagcttcaggccctcgctgaggaacaggccattgccggtggtcagctggagctggctgtctggctggttgagggtacggaggagttcctggaagccttcatggatctgagcctccggaatctccgtgaggttgaaattcaggccctccaggatttcatcgtgagtgtcagccttggtccccagggagagcattgcaaaggctgtagcgatgctcactggggagaagaagatattggtgctgttggactggtgtgccagctggcggtataggctgaaggcgaactcagccaggttgggggtgatcttgttgaaggttgggtgatcctgatcatggtgggatgtatctgtcttctgggcagcatctccctggggatcctcagccagggagacagggaccaggcagcacaggcctgccagcaggaggatgccccacgagacagaagacggcattgtcctgtggaactgagtgagcagcagcagcaatgtcccacctttcctgctctcctcaagctctcctcaagctctgtctcttctggcaggcacaggagagtggcctgaaggctggcaggaggttgccgcccctccaacctggaattcctggcagcagcagcggctaggccttcctcggaggcccgaccccctcctccttcttggttcagctcaggactctgagggttgctgcgtggaggcagtgcatgccctgggcacagtgcccagttcctgccca

SEQ ID NO: 18 - DNA, 3532 bp, Homo sapiens
tgcaagaaatgtagttctatttattctctgttctaatgggtataaacattttgttatctaacttgaacatcataccaactcaaaggcaggtcttactagcaatgactggggctcagagaggtttggcgacttcacgaaggtcacacagctgtcagggggaaaagtcagaacttggatccaggtcttcagactctcaggtctggtgtcatcctagggggcttggtgatggccatatctttaatgtatttgtggagagtgaaaggctgtcagtgagtaagcttaagagaacaggagacttgtgtgggaaacagtcggtatccattgattagactgaatcatgtagaattgctaatttcaccattttgaactatcgaaatcactatttggtatgactcaacctcatcctttaagtacacattcatgacagtgagtggttagacagtgattcctagattagtttgggatggggcagtgccttccataggacaaggccattcctggtagagacggagggagcaggctgtccttcagctaggggcccaggggacttcctggctgctgtgtcctttagcagggccttggaggatggaaggactctcctggcccttaccacaggggctattcaggaacagcctcctgccgtggcactggagctgcggtggccctctgaagactgcagggacagcaacaggcacaaagaagtcaggctgcatgtggccccagtcgggactcagaggaggaaagggaggggttgcgggggtcaatgggtgatgtgcttcctctcccatagctgaggagtccttgcaatggccttcctgagccatcagcaggcctatggccatgtgactagggaggagaagggatatagggtaatggtcttctggggcctgctgggcctggtcaagtctgaggaggagatagagaaaacaaagcagagaccctcctcttcatctggggagaagggacctgattctaaacggagatatgtgaggctttctggggcagcgatggaaggacaaggacagaataggtgtccttgttgccccatggagaatgggcttcaggaagaatctgcctcagtcattttccagaagtgcctgagaggtgcagggcccgagtctggttaggtgacagcgggtcaagaggaggacattgtcctctctcttgtgttgctgcagatgccacaaaactgggccacggcacgatcaggcagttctggggcccccaggagggcagccttggggtgggcacagccagccctggcaggatgagcaactctgggtgggggggagtgggggatgagcagggggacatgaagatgcttggtggagcctggggtcatggctggtatctggttcctcccctgtgattccttcttggggactccaagacaggacaaggaagactggagccctccagaaacagatgggcccaggtccgtaagctgaggattcagtcccccctggattcaagcccagcatgtgcctacccagccagatgctccatgaacacagttcagggggcccgaagacagcactgttacctggagcccacatacagcctcagcaggcaaagggagactcagagaaaacatgggagggatttacagtcacatgcaggcagggaccagctcaacccttctttaatgtcatccagggagggggccagggatggaggggaggggttgaggagcgagaggcagttatttttgggtgggattcaccacttttcccatgaagaggggagacttggtattttgttcaatcattaagaagacaaagggtttgttgaacttgacctcgggggggatagacatgggtatggcctctaaaaacatggccccagcagcttcagtccctttctcgtcgatggtcagcacagccttatgcacggccttggagagcttcaggggtgcctcctctgtgaccccggagaggtcagccccattgctgaagaccttagtgatgcccagttgacccaggacgctcttcagatcataggttccagtaatggacagtttgggtaaatgtaagctggcagaccttctgtcttcattttccaggaacttggtgatgatatcgtgggtgagttcattttccaggtgctgtagtttcccctcatcaggcaggaagaagatggcggtggcattgcccaggtatttcatcagcagcacccagctggacagcttcttacagtgctggatgttaaacatgcctaaacgcttcatcataggcaccttcacggtggtcacctggtccacgtggaagtcctcttcctcggtgtccttgacttcaaagggtctctcccatttgcctttaaagaagatgtaattcaccagagcaaaaactgtgtctctgtcaagctccttgaccaaatccacaattttcccttgagtacccttctccacgtaatcgttgatctgtttcttggcctcttcggtgtccccgaagttgacagtgaaggcttctgagtggtacaactttttaacatcctccaaaaacttatccactagcttcaggccctcgctgaggaacaggccattgccggtggtcagctggagctggctgtctggctggttgagggtacggaggagttcctggaagccttcatggatctgagcctccggaatctccgtgaggttgaaattcaggccctccaggatttcatcgtgagtgtcagccttggtccccagggagagcattgcaaaggctgtagcgatgctcactggggagaagaagatattggtgctgttggactggtgtgccagctggcggtataggctgaaggcgaactcagccaggttgggggtgatcttgttgaaggttgggtgatcctgatcatggtgggatgtatctgtcttctgggcagcatctccctggggatcctcagccagggagacagggaccaggcagcacaggcctgccagcaggaggatgccccacgagacagaagacggcattgtcgattcactgtcccaggtcagtggtggtgcctgaagctgaggagacagggccctgtcctcgtccgtatttaagcagtggatccagaggggcaacgggggaggctgctggctcagaaaccacagcgtcctgtgtccaaggtggagggggtggcgtgagtcagacagtctctgggagagtaccacttagctggccctctgctctcactgcagaatccttagtggctgttccactggtagcaagatctaccatttactgagtcaccccaaaatgcctgatgctgaagacttactgccgccctgtggaactgagtgagcagcagcagcaatgtcccacctttcctgctctcctcaagctctcctcaagctctgtctcttctggcaggcacaggagagtggcctgaaggctggcaggaggttgccgcccctccaacctggaattcctggcagcagcagcggctaggccttcctcggaggcccgaccccctcctccttcttggttcagctcaggactctgagggttgctgcgtggaggcagtgcatgccctgggcacagtgcccagttcctgccca

SEQ ID NO: 19 - DNA, 3340 bp, Homo sapiens
tgcaagaaatgtagttctatttattctctgttctaatgggtataaacattttgttatctaacttgaacatcataccaactcaaaggcaggtcttactagcaatgactggggctcagagaggtttggcgacttcacgaaggtcacacagctgtcagggggaaaagtcagaacttggatccaggtcttcagactctcaggtctggtgtcatcctagggggcttggtgatggccatatctttaatgtatttgtggagagtgaaaggctgtcagtgagtaagcttaagagaacaggagacttgtgtgggaaacagtcggtatccattgattagactgaatcatgtagaattgctaatttcaccattttgaactatcgaaatcactatttggtatgactcaacctcatcctttaagtacacattcatgacagtgagtggttagacagtgattcctagattagtttgggatggggcagtgccttccataggacaaggccattcctggtagagacggagggagcaggctgtccttcagctaggggcccaggggacttcctggctgctgtgtcctttagcagggccttggaggatggaaggactctcctggcccttaccacaggggctattcaggaacagcctcctgccgtggcactggagctgcggtggccctctgaagactgcagggacagcaacaggcacaaagaagtcaggctgcatgtggccccagtcgggactcagaggaggaaagggaggggttgcgggggtcaatgggtgatgtgcttcctctcccatagctgaggagtccttgcaatggccttcctgagccatcagcaggcctatggccatgtgactagggaggagaagggatatagggtaatggtcttctggggcctgctgggcctggtcaagtctgaggaggagatagagaaaacaaagcagagaccctcctcttcatctggggagaagggacctgattctaaacggagatatgtgaggctttctggggcagcgatggaaggacaaggacagaataggtgtccttgttgccccatggagaatgggcttcaggaagaatctgcctcagtcattttccagaagtgcctgagaggtgcagggcccgagtctggttaggtgacagcgggtcaagaggaggacattgtcctctctcttgtgttgctgcagatgccacaaaactgggccacggcacgatcaggcagttctggggcccccaggagggcagccttggggtgggcacagccagccctggcaggatgagcaactctgggtgggggggagtgggggatgagcagggggacatgaagatgcttggtggagcctggggtcatggctggtatctggttcctcccctgtgattccttcttggggactccaagacaggacaaggaagactggagccctccagaaacagatgggcccaggtccgtaagctgaggattcagtcccccctggattcaagcccagcatgtgcctacccagccagatgctccatgaacacagttcagggggcccgaagacagcactgttacctggagcccacatacagcctcagcaggcaaagggagactcagagaaaacatgggagggatttacagtcacatgcaggcagggaccagctcaacccttctttaatgtcatccagggagggggccagggatggaggggaggggttgaggagcgagaggcagttatttttgggtgggattcaccacttttcccatgaagaggggagacttggtattttgttcaatcattaagaagacaaagggtttgttgaacttgacctcgggggggatagacatgggtatggcctctaaaaacatggccccagcagcttcagtccctttctcgtcgatggtcagcacagccttatgcacggccttggagagcttcaggggtgcctcctctgtgaccccggagaggtcagccccattgctgaagaccttagtgatgcccagttgacccaggacgctcttcagatcataggttccagtaatggacagtttgggtaaatgtaagctggcagaccttctgtcttcattttccaggaacttggtgatgatatcgtgggtgagttcattttccaggtgctgtagtttcccctcatcaggcaggaagaagatggcggtggcattgcccaggtatttcatcagcagcacccagctggacagcttcttacagtgctggatgttaaacatgcctaaacgcttcatcataggcaccttcacggtggtcacctggtccacgtggaagtcctcttcctcggtgtccttgacttcaaagggtctctcccatttgcctttaaagaagatgtaattcaccagagcaaaaactgtgtctctgtcaagctccttgaccaaatccacaattttcccttgagtacccttctccacgtaatcgttgatctgtttcttggcctcttcggtgtccccgaagttgacagtgaaggcttctgagtggtacaactttttaacatcctccaaaaacttatccactagcttcaggccctcgctgaggaacaggccattgccggtggtcagctggagctggctgtctggctggttgagggtacggaggagttcctggaagccttcatggatctgagcctccggaatctccgtgaggttgaaattcaggccctccaggatttcatcgtgagtgtcagccttggtccccagggagagcattgcaaaggctgtagcgatgctcactggggagaagaagatattggtgctgttggactggtgtgccagctggcggtataggctgaaggcgaactcagccaggttgggggtgatcttgttgaaggttgggtgatcctgatcatggtgggatgtatctgtcttctgggcagcatctccctggggatcctcagccagggagacagggaccaggcagcacaggcctgccagcaggaggatgccccacgagacagaagacggcattgtcgattcactgtcccaggtcagtggtggtgcctgaagctgaggagacagggccctgtcctcgtccgtatttaagcagtggatccagaggggcaacgggggaggctgctgtggaactgagtgagcagcagcagcaatgtcccacctttcctgctctcctcaagctctcctcaagctctgtctcttctggcaggcacaggagagtggcctgaaggctggcaggaggttgccgcccctccaacctggaattcctggcagcagcagcggctaggccttcctcggaggcccgaccccctcctccttcttggttcagctcaggactctgagggttgctgcgtggaggcagtgcatgccctgggcacagtgcccagttcctgccca

SEQ ID NO: 20 - DNA, 3495 bp, Homo sapiens
tgcaagaaatgtagttctatttattctctgttctaatgggtataaacattttgttatctaacttgaacatcataccaactcaaaggcaggtcttactagcaatgactggggctcagagaggtttggcgacttcacgaaggtcacacagctgtcagggggaaaagtcagaacttggatccaggtcttcagactctcaggtctggtgtcatcctagggggcttggtgatggccatatctttaatgtatttgtggagagtgaaaggctgtcagtgagtaagcttaagagaacaggagacttgtgtgggaaacagtcggtatccattgattagactgaatcatgtagaattgctaatttcaccattttgaactatcgaaatcactatttggtatgactcaacctcatcctttaagtacacattcatgacagtgagtggttagacagtgattcctagattagtttgggatggggcagtgccttccataggacaaggccattcctggtagagacggagggagcaggctgtccttcagctaggggcccaggggacttcctggctgctgtgtcctttagcagggccttggaggatggaaggactctcctggcccttaccacaggggctattcaggaacagcctcctgccgtggcactggagctgcggtggccctctgaagactgcagggacagcaacaggcacaaagaagtcaggctgcatgtggccccagtcgggactcagaggaggaaagggaggggttgcgggggtcaatgggtgatgtgcttcctctcccatagctgaggagtccttgcaatggccttcctgagccatcagcaggcctatggccatgtgactagggaggagaagggatatagggtaatggtcttctggggcctgctgggcctggtcaagtctgaggaggagatagagaaaacaaagcagagaccctcctcttcatctggggagaagggacctgattctaaacggagatatgtgaggctttctggggcagcgatggaaggacaaggacagaataggtgtccttgttgccccatggagaatgggcttcaggaagaatctgcctcagtcattttccagaagtgcctgagaggtgcagggcccgagtctggttaggtgacagcgggtcaagaggaggacattgtcctctctcttgtgttgctgcagatgccacaaaactgggccacggcacgatcaggcagttctggggcccccaggagggcagccttggggtgggcacagccagccctggcaggatgagcaactctgggtgggggggagtgggggatgagcagggggacatgaagatgcttggtggagcctggggtcatggctggtatctggttcctcccctgtgattccttcttggggactccaagacaggacaaggaagactggagccctccagaaacagatgggcccaggtccgtaagctgaggattcagtcccccctggattcaagcccagcatgtgcctacccagccagatgctccatgaacacagttcagggggcccgaagacagcactgttacctggagcccacatacagcctcagcaggcaaagggagactcagagaaaacatgggagggatttacagtcacatgcaggcagggaccagctcaacccttctttaatgtcatccagggagggggccagggatggaggggaggggttgaggagcgagaggcagttatttttgggtgggattcaccacttttcccatgaagaggggagacttggtattttgttcaatcattaagaagacaaagggtttgttgaacttgacctcgggggggatagacatgggtatggcctctaaaaacatggccccagcagcttcagtccctttctcgtcgatggtcagcacagccttatgcacggccttggagagcttcaggggtgcctcctctgtgaccccggagaggtcagccccattgctgaagaccttagtgatgcccagttgacccaggacgctcttcagatcataggttccagtaatggacagtttgggtaaatgtaagctggcagaccttctgtcttcattttccaggaacttggtgatgatatcgtgggtgagttcattttccaggtgctgtagtttcccctcatcaggcaggaagaagatggcggtggcattgcccaggtatttcatcagcagcacccagctggacagcttcttacagtgctggatgttaaacatgcctaaacgcttcatcataggcaccttcacggtggtcacctggtccacgtggaagtcctcttcctcggtgtccttgacttcaaagggtctctcccatttgcctttaaagaagatgtaattcaccagagcaaaaactgtgtctctgtcaagctccttgaccaaatccacaattttcccttgagtacccttctccacgtaatcgttgatctgtttcttggcctcttcggtgtccccgaagttgacagtgaaggcttctgagtggtacaactttttaacatcctccaaaaacttatccactagcttcaggccctcgctgaggaacaggccattgccggtggtcagctggagctggctgtctggctggttgagggtacggaggagttcctggaagccttcatggatctgagcctccggaatctccgtgaggttgaaattcaggccctccaggatttcatcgtgagtgtcagccttggtccccagggagagcattgcaaaggctgtagcgatgctcactggggagaagaagatattggtgctgttggactggtgtgccagctggcggtataggctgaaggcgaactcagccaggttgggggtgatcttgttgaaggttgggtgatcctgatcatggtgggatgtatctgtcttctgggcagcatctccctggggatcctcagccagggagacagggaccaggcagcacaggcctgccagcaggaggatgccccacgagacagaagacggcattgtcgattcactgtcccaggtcagtggtggtgcctgaagctgaggagacagggccctgtcctcgtccgtatttaagcagtggatccagaggggcaacgggggaggctgctggctcagaaaccacagcgtcctgtgtccaaggtggagggggtggcgtgagtcagacagtctctgggagagtaccacttagctggccctctgctctcactgcagaatccttagtggctgttccactggtagcaagatctaccatttactgagtcaccccaaaatgcctgatgctgaagacttactgccgccctttcctgctctcctcaagctctcctcaagctctgtctcttctggcaggcacaggagagtggcctgaaggctggcaggaggttgccgcccctccaacctggaattcctggcagcagcagcggctaggccttcctcggaggcccgaccccctcctccttcttggttcagctcaggactctgagggttgctgcgtggaggcagtgcatgccctgggcacagtgcccagttcctgccca

SEQ ID NO: 21 - DNA, 3492 bp, Homo sapiens
tgcaagaaatgtagttctatttattctctgttctaatgggtataaacattttgttatctaacttgaacatcataccaactcaaaggcaggtcttactagcaatgactggggctcagagaggtttggcgacttcacgaaggtcacacagctgtcagggggaaaagtcagaacttggatccaggtcttcagactctcaggtctggtgtcatcctagggggcttggtgatggccatatctttaatgtatttgtggagagtgaaaggctgtcagtgagtaagcttaagagaacaggagacttgtgtgggaaacagtcggtatccattgattagactgaatcatgtagaattgctaatttcaccattttgaactatcgaaatcactatttggtatgactcaacctcatcctttaagtacacattcatgacagtgagtggttagacagtgattcctagattagtttgggatggggcagtgccttccataggacaaggccattcctggtagagacggagggagcaggctgtccttcagctaggggcccaggggacttcctggctgctgtgtcctttagcagggccttggaggatggaaggactctcctggcccttaccacaggggctattcaggaacagcctcctgccgtggcactggagctgcggtggccctctgaagactgcagggacagcaacaggcacaaagaagtcaggctgcatgtggccccagtcgggactcagaggaggaaagggaggggttgcgggggtcaatgggtgatgtgcttcctctcccatagctgaggagtccttgcaatggccttcctgagccatcagcaggcctatggccatgtgactagggaggagaagggatatagggtaatggtcttctggggcctgctgggcctggtcaagtctgaggaggagatagagaaaacaaagcagagaccctcctcttcatctggggagaagggacctgattctaaacggagatatgtgaggctttctggggcagcgatggaaggacaaggacagaataggtgtccttgttgccccatggagaatgggcttcaggaagaatctgcctcagtcattttccagaagtgcctgagaggtgcagggcccgagtctggttaggtgacagcgggtcaagaggaggacattgtcctctctcttgtgttgctgcagatgccacaaaactgggccacggcacgatcaggcagttctggggcccccaggagggcagccttggggtgggcacagccagccctggcaggatgagcaactctgggtgggggggagtgggggatgagcagggggacatgaagatgcttggtggagcctggggtcatggctggtatctggttcctcccctgtgattccttcttggggactccaagacaggacaaggaagactggagccctccagaaacagatgggcccaggtccgtaagctgaggattcagtcccccctggattcaagcccagcatgtgcctacccagccagatgctccatgaacacagttcagggggcccgaagacagcactgttacctggagcccacatacagcctcagcaggcaaagggagactcagagaaaacatgggagggatttacagtcacatgcaggcagggaccagctcaacccttctttaatgtcatccagggagggggccagggatggaggggaggggttgaggagcgagaggcagttatttttgggtgggattcaccacttttcccatgaagaggggagacttggtattttgttcaatcattaagaagacaaagggtttgttgaacttgacctcgggggggatagacatgggtatggcctctaaaaacatggccccagcagcttcagtccctttctcgtcgatggtcagcacagccttatgcacggccttggagagcttcaggggtgcctcctctgtgaccccggagaggtcagccccattgctgaagaccttagtgatgcccagttgacccaggacgctcttcagatcataggttccagtaatggacagtttgggtaaatgtaagctggcagaccttctgtcttcattttccaggaacttggtgatgatatcgtgggtgagttcattttccaggtgctgtagtttcccctcatcaggcaggaagaagatggcggtggcattgcccaggtatttcatcagcagcacccagctggacagcttcttacagtgctggatgttaaacatgcctaaacgcttcatcataggcaccttcacggtggtcacctggtccacgtggaagtcctcttcctcggtgtccttgacttcaaagggtctctcccatttgcctttaaagaagatgtaattcaccagagcaaaaactgtgtctctgtcaagctccttgaccaaatccacaattttcccttgagtacccttctccacgtaatcgttgatctgtttcttggcctcttcggtgtccccgaagttgacagtgaaggcttctgagtggtacaactttttaacatcctccaaaaacttatccactagcttcaggccctcgctgaggaacaggccattgccggtggtcagctggagctggctgtctggctggttgagggtacggaggagttcctggaagccttcatggatctgagcctccggaatctccgtgaggttgaaattcaggccctccaggatttcatcgtgagtgtcagccttggtccccagggagagcattgcaaaggctgtagcgatgctcactggggagaagaagatattggtgctgttggactggtgtgccagctggcggtataggctgaaggcgaactcagccaggttgggggtgatcttgttgaaggttgggtgatcctgatcatggtgggatgtatctgtcttctgggcagcatctccctggggatcctcagccagggagacagggaccaggcagcacaggcctgccagcaggaggatgccccacgagacagaagacggcattgtcgattcactgtcccaggtcagtggtggtgcctgaagctgaggagacagggccctgtcctcgtccgtatttaagcagtggatccagaggggcaacgggggaggctggctcagaaaccacagcgtcctgtgtccaaggtggagggggtggcgtgagtcagacagtctctgggagagtaccacttagctggccctctgctctcactgcagaatccttagtggctgttccactggtagcaagatctaccatttactgagtcaccccaaaatgcctgatgctgaagacttactgccgccctttcctgctctcctcaagctctcctcaagctctgtctcttctggcaggcacaggagagtggcctgaaggctggcaggaggttgccgcccctccaacctggaattcctggcagcagcagcggctaggccttcctcggaggcccgaccccctcctccttcttggttcagctcaggactctgagggttgctgcgtggaggcagtgcatgccctgggcacagtgcccagttcctgccca

SEQ ID NO: 22 - DNA, 3510 bp, Homo sapiens
tgcaagaaatgtagttctatttattctctgttctaatgggtataaacattttgttatctaacttgaacatcataccaactcaaaggcaggtcttactagcaatgactggggctcagagaggtttggcgacttcacgaaggtcacacagctgtcagggggaaaagtcagaacttggatccaggtcttcagactctcaggtctggtgtcatcctagggggcttggtgatggccatatctttaatgtatttgtggagagtgaaaggctgtcagtgagtaagcttaagagaacaggagacttgtgtgggaaacagtcggtatccattgattagactgaatcatgtagaattgctaatttcaccattttgaactatcgaaatcactatttggtatgactcaacctcatcctttaagtacacattcatgacagtgagtggttagacagtgattcctagattagtttgggatggggcagtgccttccataggacaaggccattcctggtagagacggagggagcaggctgtccttcagctaggggcccaggggacttcctggctgctgtgtcctttagcagggccttggaggatggaaggactctcctggcccttaccacaggggctattcaggaacagcctcctgccgtggcactggagctgcggtggccctctgaagactgcagggacagcaacaggcacaaagaagtcaggctgcatgtggccccagtcgggactcagaggaggaaagggaggggttgcgggggtcaatgggtgatgtgcttcctctcccatagctgaggagtccttgcaatggccttcctgagccatcagcaggcctatggccatgtgactagggaggagaagggatatagggtaatggtcttctggggcctgctgggcctggtcaagtctgaggaggagatagagaaaacaaagcagagaccctcctcttcatctggggagaagggacctgattctaaacggagatatgtgaggctttctggggcagcgatggaaggacaaggacagaataggtgtccttgttgccccatggagaatgggcttcaggaagaatctgcctcagtcattttccagaagtgcctgagaggtgcagggcccgagtctggttaggtgacagcgggtcaagaggaggacattgtcctctctcttgtgttgctgcagatgccacaaaactgggccacggcacgatcaggcagttctggggcccccaggagggcagccttggggtgggcacagccagccctggcaggatgagcaactctgggtgggggggagtgggggatgagcagggggacatgaagatgcttggtggagcctggggtcatggctggtatctggttcctcccctgtgattccttcttggggactccaagacaggacaaggaagactggagccctccagaaacagatgggcccaggtccgtaagctgaggattcagtcccccctggattcaagcccagcatgtgcctacccagccagatgctccatgaacacagttcagggggcccgaagacagcactgttacctggagcccacatacagcctcagcaggcaaagggagactcagagaaaacatgggagggatttacagtcacatgcaggcagggaccagctcaacccttctttaatgtcatccagggagggggccagggatggaggggaggggttgaggagcgagaggcagttatttttgggtgggattcaccacttttcccatgaagaggggagacttggtattttgttcaatcattaagaagacaaagggtttgttgaacttgacctcgggggggatagacatgggtatggcctctaaaaacatggccccagcagcttcagtccctttctcgtcgatggtcagcacagccttatgcacggccttggagagcttcaggggtgcctcctctgtgaccccggagaggtcagccccattgctgaagaccttagtgatgcccagttgacccaggacgctcttcagatcataggttccagtaatggacagtttgggtaaatgtaagctggcagaccttctgtcttcattttccaggaacttggtgatgatatcgtgggtgagttcattttccaggtgctgtagtttcccctcatcaggcaggaagaagatggcggtggcattgcccaggtatttcatcagcagcacccagctggacagcttcttacagtgctggatgttaaacatgcctaaacgcttcatcataggcaccttcacggtggtcacctggtccacgtggaagtcctcttcctcggtgtccttgacttcaaagggtctctcccatttgcctttaaagaagatgtaattcaccagagcaaaaactgtgtctctgtcaagctccttgaccaaatccacaattttcccttgagtacccttctccacgtaatcgttgatctgtttcttggcctcttcggtgtccccgaagttgacagtgaaggcttctgagtggtacaactttttaacatcctccaaaaacttatccactagcttcaggccctcgctgaggaacaggccattgccggtggtcagctggagctggctgtctggctggttgagggtacggaggagttcctggaagccttcatggatctgagcctccggaatctccgtgaggttgaaattcaggccctccaggatttcatcgtgagtgtcagccttggtccccagggagagcattgcaaaggctgtagcgatgctcactggggagaagaagatattggtgctgttggactggtgtgccagctggcggtataggctgaaggcgaactcagccaggttgggggtgatcttgttgaaggttgggtgatcctgatcatggtgggatgtatctgtcttctgggcagcatctccctggggatcctcagccagggagacagggaccaggcagcacaggcctgccagcaggaggatgccccacgagacagaagacggcattgtcgattcactgtcccaggtcagtggtggtgcctgaagctgaggagacagggccctgtcctcgtccgtatttaagcagtggatccagaggggcaacgggggaggcgaaaggagtcattgtacctggctcagaaaccacagcgtcctgtgtccaaggtggagggggtggcgtgagtcagacagtctctgggagagtaccacttagctggccctctgctctcactgcagaatccttagtggctgttccactggtagcaagatctaccatttactgagtcaccccaaaatgcctgatgctgaagacttactgccgccctttcctgctctcctcaagctctcctcaagctctgtctcttctggcaggcacaggagagtggcctgaaggctggcaggaggttgccgcccctccaacctggaattcctggcagcagcagcggctaggccttcctcggaggcccgaccccctcctccttcttggttcagctcaggactctgagggttgctgcgtggaggcagtgcatgccctgggcacagtgcccagttcctgccca

SEQ ID NO: 23 - DNA, 3303 bp, Homo sapiens
tgcaagaaatgtagttctatttattctctgttctaatgggtataaacattttgttatctaacttgaacatcataccaactcaaaggcaggtcttactagcaatgactggggctcagagaggtttggcgacttcacgaaggtcacacagctgtcagggggaaaagtcagaacttggatccaggtcttcagactctcaggtctggtgtcatcctagggggcttggtgatggccatatctttaatgtatttgtggagagtgaaaggctgtcagtgagtaagcttaagagaacaggagacttgtgtgggaaacagtcggtatccattgattagactgaatcatgtagaattgctaatttcaccattttgaactatcgaaatcactatttggtatgactcaacctcatcctttaagtacacattcatgacagtgagtggttagacagtgattcctagattagtttgggatggggcagtgccttccataggacaaggccattcctggtagagacggagggagcaggctgtccttcagctaggggcccaggggacttcctggctgctgtgtcctttagcagggccttggaggatggaaggactctcctggcccttaccacaggggctattcaggaacagcctcctgccgtggcactggagctgcggtggccctctgaagactgcagggacagcaacaggcacaaagaagtcaggctgcatgtggccccagtcgggactcagaggaggaaagggaggggttgcgggggtcaatgggtgatgtgcttcctctcccatagctgaggagtccttgcaatggccttcctgagccatcagcaggcctatggccatgtgactagggaggagaagggatatagggtaatggtcttctggggcctgctgggcctggtcaagtctgaggaggagatagagaaaacaaagcagagaccctcctcttcatctggggagaagggacctgattctaaacggagatatgtgaggctttctggggcagcgatggaaggacaaggacagaataggtgtccttgttgccccatggagaatgggcttcaggaagaatctgcctcagtcattttccagaagtgcctgagaggtgcagggcccgagtctggttaggtgacagcgggtcaagaggaggacattgtcctctctcttgtgttgctgcagatgccacaaaactgggccacggcacgatcaggcagttctggggcccccaggagggcagccttggggtgggcacagccagccctggcaggatgagcaactctgggtgggggggagtgggggatgagcagggggacatgaagatgcttggtggagcctggggtcatggctggtatctggttcctcccctgtgattccttcttggggactccaagacaggacaaggaagactggagccctccagaaacagatgggcccaggtccgtaagctgaggattcagtcccccctggattcaagcccagcatgtgcctacccagccagatgctccatgaacacagttcagggggcccgaagacagcactgttacctggagcccacatacagcctcagcaggcaaagggagactcagagaaaacatgggagggatttacagtcacatgcaggcagggaccagctcaacccttctttaatgtcatccagggagggggccagggatggaggggaggggttgaggagcgagaggcagttatttttgggtgggattcaccacttttcccatgaagaggggagacttggtattttgttcaatcattaagaagacaaagggtttgttgaacttgacctcgggggggatagacatgggtatggcctctaaaaacatggccccagcagcttcagtccctttctcgtcgatggtcagcacagccttatgcacggccttggagagcttcaggggtgcctcctctgtgaccccggagaggtcagccccattgctgaagaccttagtgatgcccagttgacccaggacgctcttcagatcataggttccagtaatggacagtttgggtaaatgtaagctggcagaccttctgtcttcattttccaggaacttggtgatgatatcgtgggtgagttcattttccaggtgctgtagtttcccctcatcaggcaggaagaagatggcggtggcattgcccaggtatttcatcagcagcacccagctggacagcttcttacagtgctggatgttaaacatgcctaaacgcttcatcataggcaccttcacggtggtcacctggtccacgtggaagtcctcttcctcggtgtccttgacttcaaagggtctctcccatttgcctttaaagaagatgtaattcaccagagcaaaaactgtgtctctgtcaagctccttgaccaaatccacaattttcccttgagtacccttctccacgtaatcgttgatctgtttcttggcctcttcggtgtccccgaagttgacagtgaaggcttctgagtggtacaactttttaacatcctccaaaaacttatccactagcttcaggccctcgctgaggaacaggccattgccggtggtcagctggagctggctgtctggctggttgagggtacggaggagttcctggaagccttcatggatctgagcctccggaatctccgtgaggttgaaattcaggccctccaggatttcatcgtgagtgtcagccttggtccccagggagagcattgcaaaggctgtagcgatgctcactggggagaagaagatattggtgctgttggactggtgtgccagctggcggtataggctgaaggcgaactcagccaggttgggggtgatcttgttgaaggttgggtgatcctgatcatggtgggatgtatctgtcttctgggcagcatctccctggggatcctcagccagggagacagggaccaggcagcacaggcctgccagcaggaggatgccccacgagacagaagacggcattgtcgattcactgtcccaggtcagtggtggtgcctgaagctgaggagacagggccctgtcctcgtccgtatttaagcagtggatccagaggggcaacgggggaggctgctttcctgctctcctcaagctctcctcaagctctgtctcttctggcaggcacaggagagtggcctgaaggctggcaggaggttgccgcccctccaacctggaattcctggcagcagcagcggctaggccttcctcggaggcccgaccccctcctccttcttggttcagctcaggactctgagggttgctgcgtggaggcagtgcatgccctgggcacagtgcccagttcctgccca

SEQ ID NO: 24 - DNA, 3300 bp, Homo sapiens
tgcaagaaatgtagttctatttattctctgttctaatgggtataaacattttgttatctaacttgaacatcataccaactcaaaggcaggtcttactagcaatgactggggctcagagaggtttggcgacttcacgaaggtcacacagctgtcagggggaaaagtcagaacttggatccaggtcttcagactctcaggtctggtgtcatcctagggggcttggtgatggccatatctttaatgtatttgtggagagtgaaaggctgtcagtgagtaagcttaagagaacaggagacttgtgtgggaaacagtcggtatccattgattagactgaatcatgtagaattgctaatttcaccattttgaactatcgaaatcactatttggtatgactcaacctcatcctttaagtacacattcatgacagtgagtggttagacagtgattcctagattagtttgggatggggcagtgccttccataggacaaggccattcctggtagagacggagggagcaggctgtccttcagctaggggcccaggggacttcctggctgctgtgtcctttagcagggccttggaggatggaaggactctcctggcccttaccacaggggctattcaggaacagcctcctgccgtggcactggagctgcggtggccctctgaagactgcagggacagcaacaggcacaaagaagtcaggctgcatgtggccccagtcgggactcagaggaggaaagggaggggttgcgggggtcaatgggtgatgtgcttcctctcccatagctgaggagtccttgcaatggccttcctgagccatcagcaggcctatggccatgtgactagggaggagaagggatatagggtaatggtcttctggggcctgctgggcctggtcaagtctgaggaggagatagagaaaacaaagcagagaccctcctcttcatctggggagaagggacctgattctaaacggagatatgtgaggctttctggggcagcgatggaaggacaaggacagaataggtgtccttgttgccccatggagaatgggcttcaggaagaatctgcctcagtcattttccagaagtgcctgagaggtgcagggcccgagtctggttaggtgacagcgggtcaagaggaggacattgtcctctctcttgtgttgctgcagatgccacaaaactgggccacggcacgatcaggcagttctggggcccccaggagggcagccttggggtgggcacagccagccctggcaggatgagcaactctgggtgggggggagtgggggatgagcagggggacatgaagatgcttggtggagcctggggtcatggctggtatctggttcctcccctgtgattccttcttggggactccaagacaggacaaggaagactggagccctccagaaacagatgggcccaggtccgtaagctgaggattcagtcccccctggattcaagcccagcatgtgcctacccagccagatgctccatgaacacagttcagggggcccgaagacagcactgttacctggagcccacatacagcctcagcaggcaaagggagactcagagaaaacatgggagggatttacagtcacatgcaggcagggaccagctcaacccttctttaatgtcatccagggagggggccagggatggaggggaggggttgaggagcgagaggcagttatttttgggtgggattcaccacttttcccatgaagaggggagacttggtattttgttcaatcattaagaagacaaagggtttgttgaacttgacctcgggggggatagacatgggtatggcctctaaaaacatggccccagcagcttcagtccctttctcgtcgatggtcagcacagccttatgcacggccttggagagcttcaggggtgcctcctctgtgaccccggagaggtcagccccattgctgaagaccttagtgatgcccagttgacccaggacgctcttcagatcataggttccagtaatggacagtttgggtaaatgtaagctggcagaccttctgtcttcattttccaggaacttggtgatgatatcgtgggtgagttcattttccaggtgctgtagtttcccctcatcaggcaggaagaagatggcggtggcattgcccaggtatttcatcagcagcacccagctggacagcttcttacagtgctggatgttaaacatgcctaaacgcttcatcataggcaccttcacggtggtcacctggtccacgtggaagtcctcttcctcggtgtccttgacttcaaagggtctctcccatttgcctttaaagaagatgtaattcaccagagcaaaaactgtgtctctgtcaagctccttgaccaaatccacaattttcccttgagtacccttctccacgtaatcgttgatctgtttcttggcctcttcggtgtccccgaagttgacagtgaaggcttctgagtggtacaactttttaacatcctccaaaaacttatccactagcttcaggccctcgctgaggaacaggccattgccggtggtcagctggagctggctgtctggctggttgagggtacggaggagttcctggaagccttcatggatctgagcctccggaatctccgtgaggttgaaattcaggccctccaggatttcatcgtgagtgtcagccttggtccccagggagagcattgcaaaggctgtagcgatgctcactggggagaagaagatattggtgctgttggactggtgtgccagctggcggtataggctgaaggcgaactcagccaggttgggggtgatcttgttgaaggttgggtgatcctgatcatggtgggatgtatctgtcttctgggcagcatctccctggggatcctcagccagggagacagggaccaggcagcacaggcctgccagcaggaggatgccccacgagacagaagacggcattgtcgattcactgtcccaggtcagtggtggtgcctgaagctgaggagacagggccctgtcctcgtccgtatttaagcagtggatccagaggggcaacgggggaggctttcctgctctcctcaagctctcctcaagctctgtctcttctggcaggcacaggagagtggcctgaaggctggcaggaggttgccgcccctccaacctggaattcctggcagcagcagcggctaggccttcctcggaggcccgaccccctcctccttcttggttcagctcaggactctgagggttgctgcgtggaggcagtgcatgccctgggcacagtgcccagttcctgccca

SEQ ID NO: 25 - protein, 16 aa, Unknown
  Description of Unknown: Exemplary hydrophobic membrane translocation peptide
AAVALLPAVLLALLAP

SEQ ID NO: 26 - protein, 11 aa, Unknown
  Description of Unknown: Exemplary hydrophobic membrane translocation analogue peptide
AALLPVLLAAP

SEQ ID NO: 27 - protein, 13 aa, Human immunodeficiency virus
GRKKRRQRRRPPQ

SEQ ID NO: 28 - protein, 16 aa, Drosophila sp.
RQIKIWFQNRRMKWKK

SEQ ID NO: 29 - RNA, 19 nt, Homo sapiens
cuggcacaccaguccaaca

SEQ ID NO: 30 - RNA, 19 nt, Homo sapiens
aguccaacagcaccaauau

SEQ ID NO: 31 - RNA, 19 nt, Homo sapiens
uccaacagcaccaauaucu

SEQ ID NO: 32 - RNA, 19 nt, Homo sapiens
ccaacagcaccaauaucuu

SEQ ID NO: 33 - RNA, 19 nt, Homo sapiens
aacagcaccaauaucuucu

SEQ ID NO: 34 - RNA, 19 nt, Homo sapiens
cuccccagugagcaucgcu

SEQ ID NO: 35 - RNA, 19 nt, Homo sapiens
cccagugagcaucgcuaca

SEQ ID NO: 36 - RNA, 19 nt, Homo sapiens
gugagcaucgcuacagccu

SEQ ID NO: 37 - RNA, 19 nt, Homo sapiens
ugagcaucgcuacagccuu

SEQ ID NO: 38 - RNA, 19 nt, Homo sapiens
gagcaucgcuacagccuuu

SEQ ID NO: 39 - RNA, 19 nt, Homo sapiens
caucgcuacagccuuugca

SEQ ID NO: 40 - RNA, 19 nt, Homo sapiens
cuacagccuuugcaaugcu

SEQ ID NO: 41 - RNA, 19 nt, Homo sapiens
ggaccaaggcugacacuca

SEQ ID NO: 42 - RNA, 19 nt, Homo sapiens
auccuggagggccugaauu

SEQ ID NO: 43 - RNA, 19 nt, Homo sapiens
uccuggagggccugaauuu

SEQ ID NO: 44 - RNA, 19 nt, Homo sapiens
uggauaaguuuuuggagga

SEQ ID NO: 45 - RNA, 19 nt, Homo sapiens
ggauaaguuuuuggaggau

SEQ ID NO: 46 - RNA, 19 nt, Homo sapiens
gacaccgaagaggccaaga

SEQ ID NO: 47 - RNA, 19 nt, Homo sapiens
acaccgaagaggccaagaa

SEQ ID NO: 48 - RNA, 19 nt, Homo sapiens
caccgaagaggccaagaaa

SEQ ID NO: 49 - RNA, 19 nt, Homo sapiens
aagaggccaagaaacagau

SEQ ID NO: 50 - RNA, 19 nt, Homo sapiens
gaggccaagaaacagauca

SEQ ID NO: 51 - RNA, 19 nt, Homo sapiens
auuuggucaaggagcuuga

SEQ ID NO: 52 - RNA, 19 nt, Homo sapiens
ggucaaggagcuugacaga

SEQ ID NO: 53 - RNA, 19 nt, Homo sapiens
ggagcuugacagagacaca

SEQ ID NO: 54 - RNA, 19 nt, Homo sapiens
agcuugacagagacacagu

SEQ ID NO: 55 - RNA, 19 nt, Homo sapiens
acaguuuuugcucugguga

SEQ ID NO: 56 - RNA, 19 nt, Homo sapiens
caguuuuugcucuggugaa

SEQ ID NO: 57 - RNA, 19 nt, Homo sapiens
uuugcucuggugaauuaca

SEQ ID NO: 58 - RNA, 19 nt, Homo sapiens
uugcucuggugaauuacau

SEQ ID NO: 59 - RNA, 19 nt, Homo sapiens
uacaucuucuuuaaaggca

SEQ ID NO: 60 - RNA, 19 nt, Homo sapiens
aaugggagagacccuuuga

SEQ ID NO: 61 - RNA, 19 nt, Homo sapiens
aggaagaggacuuccacgu

SEQ ID NO: 62 - RNA, 19 nt, Homo sapiens
cguuuaggcauguuuaaca

SEQ ID NO: 63 - RNA, 19 nt, Homo sapiens
guuuaggcauguuuaacau

SEQ ID NO: 64 - RNA, 19 nt, Homo sapiens
ugggugcugcugaugaaau

SEQ ID NO: 65 - RNA, 19 nt, Homo sapiens
uuccugccugaugagggga

SEQ ID NO: 66 - RNA, 19 nt, Homo sapiens
ccugccugaugaggggaaa

SEQ ID NO: 67 - RNA, 19 nt, Homo sapiens
agcaccuggaaaaugaacu

SEQ ID NO: 68 - RNA, 19 nt, Homo sapiens
uggaaaaugaacucaccca

SEQ ID NO: 69 - RNA, 19 nt, Homo sapiens
ccauuacuggaaccuauga

SEQ ID NO: 70 - RNA, 19 nt, Homo sapiens
cauuacuggaaccuaugau

SEQ ID NO: 71 - RNA, 19 nt, Homo sapiens
uuacuggaaccuaugaucu

SEQ ID NO: 72 - RNA, 19 nt, Homo sapiens
acuggaaccuaugaucuga

SEQ ID NO: 73 - RNA, 19 nt, Homo sapiens
uguuggacuggugugccag

SEQ ID NO: 74 - RNA, 19 nt, Homo sapiens
auauuggugcuguuggacu

SEQ ID NO: 75 - RNA, 19 nt, Homo sapiens
agauauuggugcuguugga

SEQ ID NO: 76 - RNA, 19 nt, Homo sapiens
aagauauuggugcuguugg

SEQ ID NO: 77 - RNA, 19 nt, Homo sapiens
agaagauauuggugcuguu

SEQ ID NO: 78 - RNA, 19 nt, Homo sapiens
agcgaugcucacuggggag

SEQ ID NO: 79 - RNA, 19 nt, Homo sapiens
uguagcgaugcucacuggg

SEQ ID NO: 80 - RNA, 19 nt, Homo sapiens
aggcuguagcgaugcucac

SEQ ID NO: 81 - RNA, 19 nt, Homo sapiens
aaggcuguagcgaugcuca

SEQ ID NO: 82 - RNA, 19 nt, Homo sapiens
aaaggcuguagcgaugcuc

SEQ ID NO: 83 - RNA, 19 nt, Homo sapiens
ugcaaaggcuguagcgaug

SEQ ID NO: 84 - RNA, 19 nt, Homo sapiens
agcauugcaaaggcuguag

SEQ ID NO: 85 - RNA, 19 nt, Homo sapiens
ugagugucagccuuggucc

SEQ ID NO: 86 - RNA, 19 nt, Homo sapiens
aauucaggcccuccaggau

SEQ ID NO: 87 - RNA, 19 nt, Homo sapiens
aaauucaggcccuccagga

SEQ ID NO: 88 - RNA, 19 nt, Homo sapiens
uccuccaaaaacuuaucca

SEQ ID NO: 89 - RNA, 19 nt, Homo sapiens
auccuccaaaaacuuaucc

SEQ ID NO: 90 - RNA, 19 nt, Homo sapiens
ucuuggccucuucgguguc

SEQ ID NO: 91 - RNA, 19 nt, Homo sapiens
uucuuggccucuucggugu

SEQ ID NO: 92 - RNA, 19 nt, Homo sapiens
uuucuuggccucuucggug

SEQ ID NO: 93 - RNA, 19 nt, Homo sapiens
aucuguuucuuggccucuu

SEQ ID NO: 94 - RNA, 19 nt, Homo sapiens
ugaucuguuucuuggccuc

SEQ ID NO: 95 - RNA, 19 nt, Homo sapiens
ucaagcuccuugaccaaau

SEQ ID NO: 96 - RNA, 19 nt, Homo sapiens
ucugucaagcuccuugacc

SEQ ID NO: 97 - RNA, 19 nt, Homo sapiens
ugugucucugucaagcucc

SEQ ID NO: 98 - RNA, 19 nt, Homo sapiens
acugugucucugucaagcu

SEQ ID NO: 99 - RNA, 19 nt, Homo sapiens
ucaccagagcaaaaacugu

SEQ ID NO: 100 - RNA, 19 nt, Homo sapiens
uucaccagagcaaaaacug

SEQ ID NO: 101 - RNA, 19 nt, Homo sapiens
uguaauucaccagagcaaa

SEQ ID NO: 102 - RNA, 19 nt, Homo sapiens
auguaauucaccagagcaa

SEQ ID NO: 103 - RNA, 19 nt, Homo sapiens
ugccuuuaaagaagaugua

SEQ ID NO: 104 - RNA, 19 nt, Homo sapiens
ucaaagggucucucccauu

SEQ ID NO: 105 - RNA, 19 nt, Homo sapiens
acguggaaguccucuuccu

SEQ ID NO: 106 - RNA, 19 nt, Homo sapiens
uguuaaacaugccuaaacg

SEQ ID NO: 107 - RNA, 19 nt, Homo sapiens
auguuaaacaugccuaaac

SEQ ID NO: 108 - RNA, 19 nt, Homo sapiens
auuucaucagcagcaccca

SEQ ID NO: 109 - RNA, 19 nt, Homo sapiens
uccccucaucaggcaggaa

SEQ ID NO: 110 - RNA, 19 nt, Homo sapiens
uuuccccucaucaggcagg

SEQ ID NO: 111 - RNA, 19 nt, Homo sapiens
aguucauuuuccaggugcu

SEQ ID NO: 112 - RNA, 19 nt, Homo sapiens
ugggugaguucauuuucca

SEQ ID NO: 113 - RNA, 19 nt, Homo sapiens
ucauagguuccaguaaugg

SEQ ID NO: 114 - RNA, 19 nt, Homo sapiens
aucauagguuccaguaaug

SEQ ID NO: 115 - RNA, 19 nt, Homo sapiens
agaucauagguuccaguaa

SEQ ID NO: 116 - RNA, 19 nt, Homo sapiens
ucagaucauagguuccagu

SEQ ID NO: 117 - DNA, 21 bp, Artificial Sequence
  Description of Artificial Sequence: Synthetic oligonucleotide
  Description of Combined DNA/RNA Molecule: Synthetic oligonucleotide
cuggcacaccaguccaacatt

SEQ ID NO: 118 - DNA, 21 bp, Artificial Sequence
  Description of Artificial Sequence: Synthetic oligonucleotide
  Description of Combined DNA/RNA Molecule: Synthetic oligonucleotide
aguccaacagcaccaauautt

SEQ ID NO: 119 - DNA, 21 bp, Artificial Sequence
  Description of Artificial Sequence: Synthetic oligonucleotide
  Description of Combined DNA/RNA Molecule: Synthetic oligonucleotide
uccaacagcaccaauaucutt

SEQ ID NO: 120 - DNA, 21 bp, Artificial Sequence
  Description of Artificial Sequence: Synthetic oligonucleotide
  Description of Combined DNA/RNA Molecule: Synthetic oligonucleotide
ccaacagcaccaauaucuutt

SEQ ID NO: 121 - DNA, 21 bp, Artificial Sequence
  Description of Artificial Sequence: Synthetic oligonucleotide
  Description of Combined DNA/RNA Molecule: Synthetic oligonucleotide
aacagcaccaauaucuucutt

SEQ ID NO: 122 - DNA, 21 bp, Artificial Sequence
  Description of Artificial Sequence: Synthetic oligonucleotide
  Description of Combined DNA/RNA Molecule: Synthetic oligonucleotide
cuccccagugagcaucgcutt

SEQ ID NO: 123 - DNA, 21 bp, Artificial Sequence
  Description of Artificial Sequence: Synthetic oligonucleotide
  Description of Combined DNA/RNA Molecule: Synthetic oligonucleotide
cccagugagcaucgcuacatt

SEQ ID NO: 124 - DNA, 21 bp, Artificial Sequence
  Description of Artificial Sequence: Synthetic oligonucleotide
  Description of Combined DNA/RNA Molecule: Synthetic oligonucleotide
gugagcaucgcuacagccutt

SEQ ID NO: 125 - DNA, 21 bp, Artificial Sequence
  Description of Artificial Sequence: Synthetic oligonucleotide
  Description of Combined DNA/RNA Molecule: Synthetic oligonucleotide
ugagcaucgcuacagccuutt

SEQ ID NO: 126 - DNA, 21 bp, Artificial Sequence
  Description of Artificial Sequence: Synthetic oligonucleotide
  Description of Combined DNA/RNA Molecule: Synthetic oligonucleotide
gagcaucgcuacagccuuutt

SEQ ID NO: 127 - DNA, 21 bp, Artificial Sequence
  Description of Artificial Sequence: Synthetic oligonucleotide
  Description of Combined DNA/RNA Molecule: Synthetic oligonucleotide
caucgcuacagccuuugcatt

SEQ ID NO: 128 - DNA, 21 bp, Artificial Sequence
  Description of Artificial Sequence: Synthetic oligonucleotide
  Description of Combined DNA/RNA Molecule: Synthetic oligonucleotide
cuacagccuuugcaaugcutt

SEQ ID NO: 129 - DNA, 21 bp, Artificial Sequence
  Description of Artificial Sequence: Synthetic oligonucleotide
  Description of Combined DNA/RNA Molecule: Synthetic oligonucleotide
ggaccaaggcugacacucatt

SEQ ID NO: 130 - DNA, 21 bp, Artificial Sequence
  Description of Artificial Sequence: Synthetic oligonucleotide
  Description of Combined DNA/RNA Molecule: Synthetic oligonucleotide
auccuggagggccugaauutt

SEQ ID NO: 131 - DNA, 21 bp, Artificial Sequence
  Description of Artificial Sequence: Synthetic oligonucleotide
  Description of Combined DNA/RNA Molecule: Synthetic oligonucleotide
uccuggagggccugaauuutt

SEQ ID NO: 132 - DNA, 21 bp, Artificial Sequence
  Description of Artificial Sequence: Synthetic oligonucleotide
  Description of Combined DNA/RNA Molecule: Synthetic oligonucleotide
uggauaaguuuuuggaggatt

SEQ ID NO: 133 - DNA, 21 bp, Artificial Sequence
  Description of Artificial Sequence: Synthetic oligonucleotide
  Description of Combined DNA/RNA Molecule: Synthetic oligonucleotide
ggauaaguuuuuggaggautt

SEQ ID NO: 134 - DNA, 21 bp, Artificial Sequence
  Description of Artificial Sequence: Synthetic oligonucleotide
  Description of Combined DNA/RNA Molecule: Synthetic oligonucleotide
gacaccgaagaggccaagatt

SEQ ID NO: 135 - DNA, 21 bp, Artificial Sequence
  Description of Artificial Sequence: Synthetic oligonucleotide
  Description of Combined DNA/RNA Molecule: Synthetic oligonucleotide
acaccgaagaggccaagaatt

SEQ ID NO: 136 - DNA, 21 bp, Artificial Sequence
  Description of Artificial Sequence: Synthetic oligonucleotide
  Description of Combined DNA/RNA Molecule: Synthetic oligonucleotide
caccgaagaggccaagaaatt

SEQ ID NO: 137 - DNA, 21 bp, Artificial Sequence
  Description of Artificial Sequence: Synthetic oligonucleotide
  Description of Combined DNA/RNA Molecule: Synthetic oligonucleotide
aagaggccaagaaacagautt

SEQ ID NO: 138 - DNA, 21 bp, Artificial Sequence
  Description of Artificial Sequence: Synthetic oligonucleotide
  Description of Combined DNA/RNA Molecule: Synthetic oligonucleotide
gaggccaagaaacagaucatt

SEQ ID NO: 139 - DNA, 21 bp, Artificial Sequence
  Description of Artificial Sequence: Synthetic oligonucleotide
  Description of Combined DNA/RNA Molecule: Synthetic oligonucleotide
auuuggucaaggagcuugatt

SEQ ID NO: 140 - DNA, 21 bp, Artificial Sequence
  Description of Artificial Sequence: Synthetic oligonucleotide
  Description of Combined DNA/RNA Molecule: Synthetic oligonucleotide
ggucaaggagcuugacagatt

SEQ ID NO: 141 - DNA, 21 bp, Artificial Sequence
  Description of Artificial Sequence: Synthetic oligonucleotide
  Description of Combined DNA/RNA Molecule: Synthetic oligonucleotide
ggagcuugacagagacacatt

SEQ ID NO: 142 - DNA, 21 bp, Artificial Sequence
  Description of Artificial Sequence: Synthetic oligonucleotide
  Description of Combined DNA/RNA Molecule: Synthetic oligonucleotide
agcuugacagagacacagutt

SEQ ID NO: 143 - DNA, 21 bp, Artificial Sequence
  Description of Artificial Sequence: Synthetic oligonucleotide
  Description of Combined DNA/RNA Molecule: Synthetic oligonucleotide
acaguuuuugcucuggugatt

SEQ ID NO: 144 - DNA, 21 bp, Artificial Sequence
  Description of Artificial Sequence: Synthetic oligonucleotide
  Description of Combined DNA/RNA Molecule: Synthetic oligonucleotide
caguuuuugcucuggugaatt

SEQ ID NO: 145 - DNA, 21 bp, Artificial Sequence
  Description of Artificial Sequence: Synthetic oligonucleotide
  Description of Combined DNA/RNA Molecule: Synthetic oligonucleotide
uuugcucuggugaauuacatt

SEQ ID NO: 146 - DNA, 21 bp, Artificial Sequence
  Description of Artificial Sequence: Synthetic oligonucleotide
  Description of Combined DNA/RNA Molecule: Synthetic oligonucleotide
uugcucuggugaauuacautt

SEQ ID NO: 147 - DNA, 21 bp, Artificial Sequence
  Description of Artificial Sequence: Synthetic oligonucleotide
  Description of Combined DNA/RNA Molecule: Synthetic oligonucleotide
uacaucuucuuuaaaggcatt

SEQ ID NO: 148 - DNA, 21 bp, Artificial Sequence
  Description of Artificial Sequence: Synthetic oligonucleotide
  Description of Combined DNA/RNA Molecule: Synthetic oligonucleotide
aaugggagagacccuuugatt

SEQ ID NO: 149 - DNA, 21 bp, Artificial Sequence
  Description of Artificial Sequence: Synthetic oligonucleotide
  Description of Combined DNA/RNA Molecule: Synthetic oligonucleotide
aggaagaggacuuccacgutt

SEQ ID NO: 150 - DNA, 21 bp, Artificial Sequence
  Description of Artificial Sequence: Synthetic oligonucleotide
  Description of Combined DNA/RNA Molecule: Synthetic oligonucleotide
cguuuaggcauguuuaacatt

SEQ ID NO: 151 - DNA, 21 bp, Artificial Sequence
  Description of Artificial Sequence: Synthetic oligonucleotide
  Description of Combined DNA/RNA Molecule: Synthetic oligonucleotide
guuuaggcauguuuaacautt

SEQ ID NO: 152 - DNA, 21 bp, Artificial Sequence
  Description of Artificial Sequence: Synthetic oligonucleotide
  Description of Combined DNA/RNA Molecule: Synthetic oligonucleotide
ugggugcugcugaugaaautt

SEQ ID NO: 153 - DNA, 21 bp, Artificial Sequence
  Description of Artificial Sequence: Synthetic oligonucleotide
  Description of Combined DNA/RNA Molecule: Synthetic oligonucleotide
uuccugccugaugaggggatt

SEQ ID NO: 154 - DNA, 21 bp, Artificial Sequence
  Description of Artificial Sequence: Synthetic oligonucleotide
  Description of Combined DNA/RNA Molecule: Synthetic oligonucleotide
ccugccugaugaggggaaatt

SEQ ID NO: 155 - DNA, 21 bp, Artificial Sequence
  Description of Artificial Sequence: Synthetic oligonucleotide
  Description of Combined DNA/RNA Molecule: Synthetic oligonucleotide
agcaccuggaaaaugaacutt

SEQ ID NO: 156 - DNA, 21 bp, Artificial Sequence
  Description of Artificial Sequence: Synthetic oligonucleotide
  Description of Combined DNA/RNA Molecule: Synthetic oligonucleotide
uggaaaaugaacucacccatt

SEQ ID NO: 157 - DNA, 21 bp, Artificial Sequence
  Description of Artificial Sequence: Synthetic oligonucleotide
  Description of Combined DNA/RNA Molecule: Synthetic oligonucleotide
ccauuacuggaaccuaugatt

SEQ ID NO: 158 - DNA, 21 bp, Artificial Sequence
  Description of Artificial Sequence: Synthetic oligonucleotide
  Description of Combined DNA/RNA Molecule: Synthetic oligonucleotide
cauuacuggaaccuaugautt

SEQ ID NO: 159 - DNA, 21 bp, Artificial Sequence
  Description of Artificial Sequence: Synthetic oligonucleotide
  Description of Combined DNA/RNA Molecule: Synthetic oligonucleotide
uuacuggaaccuaugaucutt

SEQ ID NO: 160 - DNA, 21 bp, Artificial Sequence
  Description of Artificial Sequence: Synthetic oligonucleotide
  Description of Combined DNA/RNA Molecule: Synthetic oligonucleotide
acuggaaccuaugaucugatt

SEQ ID NO: 161 - DNA, 21 bp, Artificial Sequence
  Description of Artificial Sequence: Synthetic oligonucleotide
  Description of Combined DNA/RNA Molecule: Synthetic oligonucleotide
uguuggacuggugugccagtt

SEQ ID NO: 162 - DNA, 21 bp, Artificial Sequence
  Description of Artificial Sequence: Synthetic oligonucleotide
  Description of Combined DNA/RNA Molecule: Synthetic oligonucleotide
auauuggugcuguuggacutt

SEQ ID NO: 163 - DNA, 21 bp, Artificial Sequence
  Description of Artificial Sequence: Synthetic oligonucleotide
  Description of Combined DNA/RNA Molecule: Synthetic oligonucleotide
agauauuggugcuguuggatt

SEQ ID NO: 164 - DNA, 21 bp, Artificial Sequence
  Description of Artificial Sequence: Synthetic oligonucleotide
  Description of Combined DNA/RNA Molecule: Synthetic oligonucleotide
aagauauuggugcuguuggtt

SEQ ID NO: 165 - DNA, 21 bp, Artificial Sequence
  Description of Artificial Sequence: Synthetic oligonucleotide
  Description of Combined DNA/RNA Molecule: Synthetic oligonucleotide
agaagauauuggugcuguutt

SEQ ID NO: 166 - DNA, 21 bp, Artificial Sequence
  Description of Artificial Sequence: Synthetic oligonucleotide
  Description of Combined DNA/RNA Molecule: Synthetic oligonucleotide
agcgaugcucacuggggagtt

SEQ ID NO: 167 - DNA, 21 bp, Artificial Sequence
  Description of Artificial Sequence: Synthetic oligonucleotide
  Description of Combined DNA/RNA Molecule: Synthetic oligonucleotide
uguagcgaugcucacugggtt

SEQ ID NO: 168 - DNA, 21 bp, Artificial Sequence
  Description of Artificial Sequence: Synthetic oligonucleotide
  Description of Combined DNA/RNA Molecule: Synthetic oligonucleotide
aggcuguagcgaugcucactt

SEQ ID NO: 169 - DNA, 21 bp, Artificial Sequence
  Description of Artificial Sequence: Synthetic oligonucleotide
  Description of Combined DNA/RNA Molecule: Synthetic oligonucleotide
aaggcuguagcgaugcucatt

SEQ ID NO: 170 - DNA, 21 bp, Artificial Sequence
  Description of Artificial Sequence: Synthetic oligonucleotide
  Description of Combined DNA/RNA Molecule: Synthetic oligonucleotide
aaaggcuguagcgaugcuctt

SEQ ID NO: 171 - DNA, 21 bp, Artificial Sequence
  Description of Artificial Sequence: Synthetic oligonucleotide
  Description of Combined DNA/RNA Molecule: Synthetic oligonucleotide
ugcaaaggcuguagcgaugtt

SEQ ID NO: 172 - DNA, 21 bp, Artificial Sequence
  Description of Artificial Sequence: Synthetic oligonucleotide
  Description of Combined DNA/RNA Molecule: Synthetic oligonucleotide
agcauugcaaaggcuguagtt

SEQ ID NO: 173 - DNA, 21 bp, Artificial Sequence
  Description of Artificial Sequence: Synthetic oligonucleotide
  Description of Combined DNA/RNA Molecule: Synthetic oligonucleotide
ugagugucagccuuggucctt

SEQ ID NO: 174 - DNA, 21 bp, Artificial Sequence
  Description of Artificial Sequence: Synthetic oligonucleotide
  Description of Combined DNA/RNA Molecule: Synthetic oligonucleotide
aauucaggcccuccaggautt

SEQ ID NO: 175 - DNA, 21 bp, Artificial Sequence
  Description of Artificial Sequence: Synthetic oligonucleotide
  Description of Combined DNA/RNA Molecule: Synthetic oligonucleotide
aaauucaggcccuccaggatt

SEQ ID NO: 176 - DNA, 21 bp, Artificial Sequence
  Description of Artificial Sequence: Synthetic oligonucleotide
  Description of Combined DNA/RNA Molecule: Synthetic oligonucleotide
uccuccaaaaacuuauccatt

SEQ ID NO: 177 - DNA, 21 bp, Artificial Sequence
  Description of Artificial Sequence: Synthetic oligonucleotide
  Description of Combined DNA/RNA Molecule: Synthetic oligonucleotide
auccuccaaaaacuuaucctt

SEQ ID NO: 178 - DNA, 21 bp, Artificial Sequence
  Description of Artificial Sequence: Synthetic oligonucleotide
  Description of Combined DNA/RNA Molecule: Synthetic oligonucleotide
ucuuggccucuucgguguctt

SEQ ID NO: 179 - DNA, 21 bp, Artificial Sequence
  Description of Artificial Sequence: Synthetic oligonucleotide
  Description of Combined DNA/RNA Molecule: Synthetic oligonucleotide
uucuuggccucuucggugutt

SEQ ID NO: 180 - DNA, 21 bp, Artificial Sequence
  Description of Artificial Sequence: Synthetic oligonucleotide
  Description of Combined DNA/RNA Molecule: Synthetic oligonucleotide
uuucuuggccucuucggugtt

SEQ ID NO: 181 - DNA, 21 bp, Artificial Sequence
  Description of Artificial Sequence: Synthetic oligonucleotide
  Description of Combined DNA/RNA Molecule: Synthetic oligonucleotide
aucuguuucuuggccucuutt

SEQ ID NO: 182 - DNA, 21 bp, Artificial Sequence
  Description of Artificial Sequence: Synthetic oligonucleotide
  Description of Combined DNA/RNA Molecule: Synthetic oligonucleotide
ugaucuguuucuuggccuctt

SEQ ID NO: 183 - DNA, 21 bp, Artificial Sequence
  Description of Artificial Sequence: Synthetic oligonucleotide
  Description of Combined DNA/RNA Molecule: Synthetic oligonucleotide
ucaagcuccuugaccaaautt

SEQ ID NO: 184 - DNA, 21 bp, Artificial Sequence
  Description of Artificial Sequence: Synthetic oligonucleotide
  Description of Combined DNA/RNA Molecule: Synthetic oligonucleotide
ucugucaagcuccuugacctt

SEQ ID NO: 185 - DNA, 21 bp, Artificial Sequence
  Description of Artificial Sequence: Synthetic oligonucleotide
  Description of Combined DNA/RNA Molecule: Synthetic oligonucleotide
ugugucucugucaagcucctt

SEQ ID NO: 186 - DNA, 21 bp, Artificial Sequence
  Description of Artificial Sequence: Synthetic oligonucleotide
  Description of Combined DNA/RNA Molecule: Synthetic oligonucleotide
acugugucucugucaagcutt

SEQ ID NO: 187 - DNA, 21 bp, Artificial Sequence
  Description of Artificial Sequence: Synthetic oligonucleotide
  Description of Combined DNA/RNA Molecule: Synthetic oligonucleotide
ucaccagagcaaaaacugutt

SEQ ID NO: 188 - DNA, 21 bp, Artificial Sequence
  Description of Artificial Sequence: Synthetic oligonucleotide
  Description of Combined DNA/RNA Molecule: Synthetic oligonucleotide
uucaccagagcaaaaacugtt

SEQ ID NO: 189 - DNA, 21 bp, Artificial Sequence
  Description of Artificial Sequence: Synthetic oligonucleotide
  Description of Combined DNA/RNA Molecule: Synthetic oligonucleotide
uguaauucaccagagcaaatt

SEQ ID NO: 190 - DNA, 21 bp, Artificial Sequence
  Description of Artificial Sequence: Synthetic oligonucleotide
  Description of Combined DNA/RNA Molecule: Synthetic oligonucleotide
auguaauucaccagagcaatt

SEQ ID NO: 191 - DNA, 21 bp, Artificial Sequence
  Description of Artificial Sequence: Synthetic oligonucleotide
  Description of Combined DNA/RNA Molecule: Synthetic oligonucleotide
ugccuuuaaagaagauguatt

SEQ ID NO: 192 - DNA, 21 bp, Artificial Sequence
  Description of Artificial Sequence: Synthetic oligonucleotide
  Description of Combined DNA/RNA Molecule: Synthetic oligonucleotide
ucaaagggucucucccauutt

SEQ ID NO: 193 - DNA, 21 bp, Artificial Sequence
  Description of Artificial Sequence: Synthetic oligonucleotide
  Description of Combined DNA/RNA Molecule: Synthetic oligonucleotide
acguggaaguccucuuccutt

SEQ ID NO: 194 - DNA, 21 bp, Artificial Sequence
  Description of Artificial Sequence: Synthetic oligonucleotide
  Description of Combined DNA/RNA Molecule: Synthetic oligonucleotide
uguuaaacaugccuaaacgtt

SEQ ID NO: 195 - DNA, 21 bp, Artificial Sequence
  Description of Artificial Sequence: Synthetic oligonucleotide
  Description of Combined DNA/RNA Molecule: Synthetic oligonucleotide
auguuaaacaugccuaaactt

SEQ ID NO: 196 - DNA, 21 bp, Artificial Sequence
  Description of Artificial Sequence: Synthetic oligonucleotide
  Description of Combined DNA/RNA Molecule: Synthetic oligonucleotide
auuucaucagcagcacccatt

SEQ ID NO: 197 - DNA, 21 bp, Artificial Sequence
  Description of Artificial Sequence: Synthetic oligonucleotide
  Description of Combined DNA/RNA Molecule: Synthetic oligonucleotide
uccccucaucaggcaggaatt

SEQ ID NO: 198 - DNA, 21 bp, Artificial Sequence
  Description of Artificial Sequence: Synthetic oligonucleotide
  Description of Combined DNA/RNA Molecule: Synthetic oligonucleotide
uuuccccucaucaggcaggtt

SEQ ID NO: 199 - DNA, 21 bp, Artificial Sequence
  Description of Artificial Sequence: Synthetic oligonucleotide
  Description of Combined DNA/RNA Molecule: Synthetic oligonucleotide
aguucauuuuccaggugcutt

SEQ ID NO: 200 - DNA, 21 bp, Artificial Sequence
  Description of Artificial Sequence: Synthetic oligonucleotide
  Description of Combined DNA/RNA Molecule: Synthetic oligonucleotide
ugggugaguucauuuuccatt

SEQ ID NO: 201 - DNA, 21 bp, Artificial Sequence
  Description of Artificial Sequence: Synthetic oligonucleotide
  Description of Combined DNA/RNA Molecule: Synthetic oligonucleotide
ucauagguuccaguaauggtt

SEQ ID NO: 202 - DNA, 21 bp, Artificial Sequence
  Description of Artificial Sequence: Synthetic oligonucleotide
  Description of Combined DNA/RNA Molecule: Synthetic oligonucleotide
aucauagguuccaguaaugtt

SEQ ID NO: 203 - DNA, 21 bp, Artificial Sequence
  Description of Artificial Sequence: Synthetic oligonucleotide
  Description of Combined DNA/RNA Molecule: Synthetic oligonucleotide
agaucauagguuccaguaatt

SEQ ID NO: 204 - DNA, 21 bp, Artificial Sequence
  Description of Artificial Sequence: Synthetic oligonucleotide
  Description of Combined DNA/RNA Molecule: Synthetic oligonucleotide
ucagaucauagguuccagutt